European Patent Application EP 4 471 121 A1, published December 4, 2024. Title: ALGAE, METHOD FOR IMPROVING GROWTH OF ALGAE IN DARK, METHOD FOR PRODUCING ALGAE WITH IMPROVED GROWTH IN DARK, DARK-ACTIVATED CRYPTOCHROME, AND POLYNUCLEOTID CODING DARK-ACTIVATED CRYPTOCHROME. Applicant: DIC Corporation. The sequence listing filed with the application follows.

SEQUENCE LISTING (88 sequences)

SEQ ID NO: 1 - skipped

SEQ ID NO: 2 - protein, 12 aa, Cyanidioschyzon merolae
  VARIANT 2: note = X can be any naturally occurring amino acid
  VARIANT 3: note = hydrophobic amino acid
  VARIANT 6..7: note = X can be any naturally occurring amino acid
  VARIANT 9..11: note = X can be any naturally occurring amino acid
  VARIANT 12: note = hydrophobic amino acid
LXXPWXXGXXXX

SEQ ID NO: 3 - protein, 12 aa, Cyanidioschyzon merolae
  VARIANT 2: note = X can be any naturally occurring amino acid
  VARIANT 3: note = hydrophobic amino acid
  VARIANT 6..7: note = X can be any naturally occurring amino acid
  VARIANT 9: note = X can be any naturally occurring amino acid
  VARIANT 10: note = basic amino acid
  VARIANT 11: note = X can be any naturally occurring amino acid
  VARIANT 12: note = X can be any naturally occurring amino acid
LXXPWXXGXXXX

SEQ ID NO: 4-6 - skipped (3 entries)

SEQ ID NO: 7 - protein, 12 aa, Cyanidioschyzon merolae
LLLPWQIGARCL

SEQ ID NO: 8 - protein, 12 aa, Cyanidioschyzon merolae
LLIPWQHGLRFL

SEQ ID NO: 9 - protein, 12 aa, Cyanidioschyzon merolae
LLLPWQIRARCL

SEQ ID NO: 10 - protein, 12 aa, Cyanidioschyzon merolae
LLIPWQHRLRFL

SEQ ID NO: 11 - DNA, 3678 bp, Cyanidioschyzon merolae
  source 1..3678: mol_type = genomic DNA
atgtcgtcgtcgagacgaccttcggttgtgtggtaccgcggccacgacctccgtgttgaggacatgccagcgttgcttgctgccgtgcagcgcggaggcccggtggtgccggtgttcatctgggcacccgaagaggacggtatgtggtgtctcggccgaccggcacgttggtggttgagtcgttccattgttgcacttgaccgacgacttcgggagctaggttgcgaaaccgggttaattctgaggcgtgcgaagtcggaaagcggcggcggcggcggcgtcgagacgacgcttctggaggtcgtgaaacgctgcggtgccgaggctgtgtactggaatcgggtctacgaccctgttgtgttacgcagagatgaggaagtgcggcggcgatggtcgaagcaccaccgcctggctgttgagtccttcaaggcggagctcctggtcgagccgtgggaggtttgtgcaacagagagcaggcccgcgagctttggggaccgtccgctcgacaccttccacgagttcatgtcagcgtggatggctatgccaccacccccagagccgttgcctgcacctaagcgaatagagccgctcattgcctcccagtcgggagatcaggggcctctgttcgctgtgcccgagtccacgatgcaaccgtcggatgtgctgcagtcgcccggcggcgaggataccgacactgaaatgggaatttggtggaaccagatacacaacttaggcagccttgaggagtactggcgccccggcgtggattgtgtagcagagcgcctgcaagacttcttgacgagtgtctttccgacgtatggggacgctcgaagacgacagcgtctccgaaacgggacatcacggctttcgccgtacctacggttcggagaattgtcaccgcggcgcctctaccacgctgttcgggcgtctgtactgcagtctgagccatcagatgcaataattcgggctgctcgaacgctcctgagaaacctctgcctccgcgagtacgcttatcatatgctattttaccgaccatcgatcctggatagaccactggtgccagaatttgatcattttccatgcaccaaggaagatgtgggccgtctcctcgaggtgtggctctcgggacgcacgggctacccactcgttgatgcggcaatgcgggaactgcaccacaccggctggttgcattcgaatctgcggtttcttgtagcttctttttttaccaagtaccttctcctgccgtggcagatcggggctcgttgcctcttcaaactattcatcgatggcgatctggcgagcaacgcgatctgctggcagtgggtgacgggctgcaactacgacgttttccccttgaattgcctcgtgaacccagtcgtgatgggcatgcgcgtagaccccgagggtgagtacgtgcgtacctggtgtccagagttgcaacagatccccagtagctacatccatgcggtgtggaaatgccctccgacgattctgcatcaggctagggttgaactgggtgtcacctatccgcgaccggttgtcgagaatcgggtagcacgtcgccgagcccgggacgcgcttcgataccttcgccaagttgtgctgaacaagcgcggctacggtgtgcgggtcccgaatacgctatcgctgaaggggactcaggaactcatgagcgattggcccattgatgaggtctacaacgtgttggattctaaacaggaagacctcttcgggctgagcgatcttggtcacgaactacctagcggaaggcagcctgagcgtcccatgcgagatagcgacgccagcatcgatgatcaggaaatagctggtgattcgatcggaggcgatcatgttggactgctcccacgggtctggtccatgagccaagacgatccgctgcacaacgtttttgatctgggcggcagtgcgagcggggcgaatggcgcgcagctggcggggccttccccgggtcttggcggcagtaacggttacgctcagggaccaggtggcggaaacggaggctcctctttgatgtacggtgtgagtgcgggcacatttgggaaccaacaaatggcgcttgtttcgagcggcatgggcatgggcagcagcggcgttggtggtggcggcggcggcggcggcggcggctccgaccgcagcatacccgaggtcgtcgtgggagctccaagtagcgtggatgaagattcctacaccgagaaactgcaccgcgtcgattcgtttcatgcactcttgtctgctggtgcaaccacgccacttgcacgcggctcgatcatggagcccactggacgagtcccgggaacaaatcctgactttatgcgcgcgcctccgacggagcatctcagtagcctgagcggcattgtagcgccaaacgccagtcatccgtcgtccgcggtgcatgtgtcgacgtcgggaagccgatcgcttgtgacggctggtggagcggcggcagccctgtcacccggccagatgatgcgcacgcccaacgcggcggttgatccaggtaccacgagcgcatcgccgctgttgctgcaccatactggtggggcgggccacggtcgaggcagttcacgaggcaccgccacgttaccggggtcacagtcgcagccgatgggtactcgatcgatgctgaacgccaacctgcccgggtctgtttttgcgttcgagtccggagaaccgggcgccatgcctcgcccagcaccgggtcattcgctgggacccgaaaccagcgtttccgcacctgcctcgtgggcgcttatcaatgagcgtccgtcgttgtcggcagctgaggatgcgagcgtgcaccggcgacccggcgcgatgccggcatcgacctcgactcggtacgataatggcgaagctgcgcggtatctagaggacagagctggacggaaacgtgcactagctgacgaaggcgtttgcaccaaccctgacttgacgatgccagagaggttccccgcggtggctgccgcgcgagttacgcagcgcttagaacatgatacagcgggcagcgtatcatctgcagcgaaaaccaagcgaagagcgtccggtgctgcagccgcaccgcaagcaccggcccagcagcgaacgcgcgatggatccgccccgaatgaggctcctgctcccggatccagcgccttgcaccatgacgcaacgcgtgcccccgctggaagccgctggctcgagcaaggcgccagtggcgaaagtctcgacgtgcgctcttcgtcggcctcgagcgaccgcacagcaccgatcacccttgagggtctgggagacgtcgagccgccccagacccggagcgaacgactcgaactgctggagcgcatccaccggagcgataacgcgtacgcccgattcgcgggtttccttctccagcactacgatatcacagagaatgtgcgccgaaaccccaagagcacggatttcgtacgtttacggaatctcaaagaccacttcaatcgatacagtgcaccaccacgggctggtcaaggtgccgctcatcgggagccgctcagaatttaccgaatcaaacaatttttcagcaaaatactgaacctggaggtcaccggcgagtgggatcgacacgcacacggcggagtgcgcggcccgtacgtgtacggcctggtgctgcgcgcggatgcgctacagcgtgccgcgccctga

SEQ ID NO: 12 - protein, 1225 aa, Cyanidioschyzon merolae
MSSSRRPSVVWYRGHDLRVEDMPALLAAVQRGGPVVPVFIWAPEEDGMWCLGRPARWWLSRSIVALDRRLRELGCETGLILRRAKSESGGGGGVETTLLEVVKRCGAEAVYWNRVYDPVVLRRDEEVRRRWSKHHRLAVESFKAELLVEPWEVCATESRPASFGDRPLDTFHEFMSAWMAMPPPPEPLPAPKRIEPLIASQSGDQGPLFAVPESTMQPSDVLQSPGGEDTDTEMGIWWNQIHNLGSLEEYWRPGVDCVAERLQDFLTSVFPTYGDARRRQRLRNGTSRLSPYLRFGELSPRRLYHAVRASVLQSEPSDAIIRAARTLLRNLCLREYAYHMLFYRPSILDRPLVPEFDHFPCTKEDVGRLLEVWLSGRTGYPLVDAAMRELHHTGWLHSNLRFLVASFFTKYLLLPWQIGARCLFKLFIDGDLASNAICWQWVTGCNYDVFPLNCLVNPVVMGMRVDPEGEYVRTWCPELQQIPSSYIHAVWKCPPTILHQARVELGVTYPRPVVENRVARRRARDALRYLRQVVLNKRGYGVRVPNTLSLKGTQELMSDWPIDEVYNVLDSKQEDLFGLSDLGHELPSGRQPERPMRDSDASIDDQEIAGDSIGGDHVGLLPRVWSMSQDDPLHNVFDLGGSASGANGAQLAGPSPGLGGSNGYAQGPGGGNGGSSLMYGVSAGTFGNQQMALVSSGMGMGSSGVGGGGGGGGGGSDRSIPEVVVGAPSSVDEDSYTEKLHRVDSFHALLSAGATTPLARGSIMEPTGRVPGTNPDFMRAPPTEHLSSLSGIVAPNASHPSSAVHVSTSGSRSLVTAGGAAAALSPGQMMRTPNAAVDPGTTSASPLLLHHTGGAGHGRGSSRGTATLPGSQSQPMGTRSMLNANLPGSVFAFESGEPGAMPRPAPGHSLGPETSVSAPASWALINERPSLSAAEDASVHRRPGAMPASTSTRYDNGEAARYLEDRAGRKRALADEGVCTNPDLTMPERFPAVAAARVTQRLEHDTAGSVSSAAKTKRRASGAAAAPQAPAQQRTRDGSAPNEAPAPGSSALHHDATRAPAGSRWLEQGASGESLDVRSSSASSDRTAPITLEGLGDVEPPQTRSERLELLERIHRSDNAYARFAGFLLQHYDITENVRRNPKSTDFVRLRNLKDHFNRYSAPPRAGQGAAHREPLRIYRIKQFFSKILNLEVTGEWDRHAHGGVRGPYVYGLVLRADALQRAAP

SEQ ID NO: 13 - DNA, 3147 bp, Cyanidioschyzon merolae
  source 1..3147: mol_type = genomic DNA
atgcccgcgtatcctccttcagaaactagtggagaggagtgtccgtggcttgctttgagcagctccccgttgctcgaagcggggcgggaggtgaacgcgcatccgccaccgggacgtacaccagcgctcgcagtggctgcagcgcagggcgcgacacagcgccccatactggtatggtaccgggggcacgacctccgaatagatgatcatgctgccttctgtgcggctgcagaaacgggtatgccggtggttcctgtgtacgtttggaacccgcaactgccgtggatgagtaaacctggcagagcagggcgctggcggctgcgagagtcgctgctggcgctggaccgggagttcgcgcaccgctacggcgaagatgcgcggctggtggttctgcaggggagcctcgtggaaagcattgtggagctggcgcgggaaacgaatgcgagcgcagtctacttcaaccgctgctacgatatcggtgccgcagaagtggaccgaacgttggaacaacgccttgctgtttggaatgttgaactcgttagcttcaaatcggaacttcttgtggagccgtgggagcttgctcaagacaacggtgagccattcaatgagtttcaccccttcatggaaaagtggctcgctttcccgaaaccgcccccacctgtagcagcgccattgaggctgcagacgctgcctggtttacggcaacgcgtttcccatgtcgagattcatgagctggagctggtctctgatctcagtccggaatggtgtgcccagatggaatgcatgtggccgcttgtcggtgagcgagcagcgtggattacgttgtcaaggtttctccgagagcgttatcccaaattcgggcgtcgagagtctcgttgtgcgctcgacggcacgagccgcctctccatgcatgttcgtttcggtgagattagcccgcggcagctgtatgcagcaatcatggctgacatcgtgtcggacgcgcctagcgcgctttccctagggaatggaataccagcgcattcgagggagcagaacggttacctggagtcgccacaccgaatcagtgcaacacctcactccatggatgctactgctattgctactgctactgctgcagttcccggttatcagccgcagcgagcgccgatgtttccgcttcgggttcaagtgaaccgaccacgaggctccagtggcacgacctactttctctacgatcatgaggatgacgacgacgacgataataataataataatggtgatgaagcagatgacaacgacgacggaggtcgtggtggtaccgatcaagcggctccaaggagcacacggcatgcgctcctgaaccgtgagcgtcacgctacagcaggcgaggcgctcgcggcaaacacacgtacccacaccgatgcagcagatgcacaacagaccatcagcgcggtgaaggcgttcctgaaaaacatgtgcctccgagaattcgcgtatcacctgctctttcacaatccacaggccttcgaagagccgctactgcccgaattccgcgcctttccttggcgctggaacgatcagagcatgctcgaggtttggcgaagcggccaaaccgggtatcccatcattgacgcagcgattcgggagttgcgtaccactggatacctgcataatcgcattcgtttcatgatcgccggcttcctgaccaagtaccttctcattccgtggcagcatggtctccgctttctttacgatcatgttctcgacggggacatagcctgtcagacgctcgggtggcagtggacggcaggctgccacaccgatgcgttcccgtttgcgtgtatcgtcaatccgatcacgtttgggctcagagaagatccccatggtgagtacgtgaagcgctgggtacccgaattggccgcactgcctacgtgttacgtccatcgtccgtggcgagcgccagcttcagtgcttgcgcaagcgggtatcgcgctgggctcttgctatgcgcatccggtggtggactcgcggacggctcgagcgcgagcactcgactccatggacctcatgcggcgtgtatttgtactgcgacaaccaacccgatccctgtggtctttaattgatctgcaacagccgcagttgtggcttgagcaatctgcatcggattcggacgattccgggatggaaacgttctctttcacgaatggaacgccatacgcacttcatgatcgcttttcaaggggctcaacgaccatcattgaggagctcgccccgaccgtcgagcacaacgctcttcagtcgctttcctatggtaaccacagtcgtcgagcattcggcattggcagtgtacatacagcagcagcgttggtgccagaaagccgacaacgacaacgacgaggctacgcgccctcctggatcgaacgtgcggacgcaggagcgtctgaagttggtgcgatgcagcctggcggacgctcttcggggtcgtcttcgcaactgagtgtagtgcgtcccgagcaactcaatgagtttctccgctgggtaactggtccagaggatgctgccgccaaccaggaacaagcatcggcaacggcaaacgagcagttgcgagcatggaatgacccgctggagcgtgtccagactgcggacattggtcgggagctctcgcctatcacgacgagtgcgcagagcgtgaccctggaaccagcgcagccacagaaacggcgacgtggaggccagcgcaatcctacgcgagcgagcatgctcggtgtagcggaacgcgaagagatattggcagcgatagcgctgcaacctaaccaaccgtttcactgcttcgcgcgcttcctgatgcagcactatcgtttcacaccgaatacggttttcggaccacatacggactttgttcgcttgcgcgcgctcaaagcagagttagctgctgcaggaacatcttgcgaggattcgacgacctccgaaaggagccgctcgtatgaacgacagaaaagccgttgcctcggtcacgttttaactgttgcgaaaatgaagcactttctgcggaatacgcttggactagaggtcactggccagtgggatcgtcgagcgcacggcggggtgcgaggtccgtacgcctacggcctcacgcgctgcccagcgagcgacgacaagcgcagatga

SEQ ID NO: 14 - protein, 1048 aa, Cyanidioschyzon merolae
MPAYPPSETSGEECPWLALSSSPLLEAGREVNAHPPPGRTPALAVAAAQGATQRPILVWYRGHDLRIDDHAAFCAAAETGMPVVPVYVWNPQLPWMSKPGRAGRWRLRESLLALDREFAHRYGEDARLVVLQGSLVESIVELARETNASAVYFNRCYDIGAAEVDRTLEQRLAVWNVELVSFKSELLVEPWELAQDNGEPFNEFHPFMEKWLAFPKPPPPVAAPLRLQTLPGLRQRVSHVEIHELELVSDLSPEWCAQMECMWPLVGERAAWITLSRFLRERYPKFGRRESRCALDGTSRLSMHVRFGEISPRQLYAAIMADIVSDAPSALSLGNGIPAHSREQNGYLESPHRISATPHSMDATAIATATAAVPGYQPQRAPMFPLRVQVNRPRGSSGTTYFLYDHEDDDDDDNNNNNGDEADDNDDGGRGGTDQAAPRSTRHALLNRERHATAGEALAANTRTHTDAADAQQTISAVKAFLKNMCLREFAYHLLFHNPQAFEEPLLPEFRAFPWRWNDQSMLEVWRSGQTGYPIIDAAIRELRTTGYLHNRIRFMIAGFLTKYLLIPWQHGLRFLYDHVLDGDIACQTLGWQWTAGCHTDAFPFACIVNPITFGLREDPHGEYVKRWVPELAALPTCYVHRPWRAPASVLAQAGIALGSCYAHPVVDSRTARARALDSMDLMRRVFVLRQPTRSLWSLIDLQQPQLWLEQSASDSDDSGMETFSFTNGTPYALHDRFSRGSTTIIEELAPTVEHNALQSLSYGNHSRRAFGIGSVHTAAALVPESRQRQRRGYAPSWIERADAGASEVGAMQPGGRSSGSSSQLSVVRPEQLNEFLRWVTGPEDAAANQEQASATANEQLRAWNDPLERVQTADIGRELSPITTSAQSVTLEPAQPQKRRRGGQRNPTRASMLGVAEREEILAAIALQPNQPFHCFARFLMQHYRFTPNTVFGPHTDFVRLRALKAELAAAGTSCEDSTTSERSRSYERQKSRCLGHVLTVAKMKHFLRNTLGLEVTGQWDRRAHGGVRGPYAYGLTRCPASDDKRR

SEQ ID NO: 15 - DNA, 3678 bp, Cyanidioschyzon merolae
  source 1..3678: mol_type = genomic DNA
atgtcgtcgtcgagacgaccttcggttgtgtggtaccgcggccacgacctccgtgttgaggacatgccagcgttgcttgctgccgtgcagcgcggaggcccggtggtgccggtgttcatctgggcacccgaagaggacggtatgtggtgtctcggccgaccggcacgttggtggttgagtcgttccattgttgcacttgaccgacgacttcgggagctaggttgcgaaaccgggttaattctgaggcgtgcgaagtcggaaagcggcggcggcggcggcgtcgagacgacgcttctggaggtcgtgaaacgctgcggtgccgaggctgtgtactggaatcgggtctacgaccctgttgtgttacgcagagatgaggaagtgcggcggcgatggtcgaagcaccaccgcctggctgttgagtccttcaaggcggagctcctggtcgagccgtgggaggtttgtgcaacagagagcaggcccgcgagctttggggaccgtccgctcgacaccttccacgagttcatgtcagcgtggatggctatgccaccacccccagagccgttgcctgcacctaagcgaatagagccgctcattgcctcccagtcgggagatcaggggcctctgttcgctgtgcccgagtccacgatgcaaccgtcggatgtgctgcagtcgcccggcggcgaggataccgacactgaaatgggaatttggtggaaccagatacacaacttaggcagccttgaggagtactggcgccccggcgtggattgtgtagcagagcgcctgcaagacttcttgacgagtgtctttccgacgtatggggacgctcgaagacgacagcgtctccgaaacgggacatcacggctttcgccgtacctacggttcggagaattgtcaccgcggcgcctctaccacgctgttcgggcgtctgtactgcagtctgagccatcagatgcaataattcgggctgctcgaacgctcctgagaaacctctgcctccgcgagtacgcttatcatatgctattttaccgaccatcgatcctggatagaccactggtgccagaatttgatcattttccatgcaccaaggaagatgtgggccgtctcctcgaggtgtggctctcgggacgcacgggctacccactcgttgatgcggcaatgcgggaactgcaccacaccggctggttgcattcgaatctgcggtttcttgtagcttctttttttaccaagtaccttctcctgccgtggcagatccgcgctcgttgcctcttcaaactattcatcgatggcgatctggcgagcaacgcgatctgctggcagtgggtgacgggctgcaactacgacgttttccccttgaattgcctcgtgaacccagtcgtgatgggcatgcgcgtagaccccgagggtgagtacgtgcgtacctggtgtccagagttgcaacagatccccagtagctacatccatgcggtgtggaaatgccctccgacgattctgcatcaggctagggttgaactgggtgtcacctatccgcgaccggttgtcgagaatcgggtagcacgtcgccgagcccgggacgcgcttcgataccttcgccaagttgtgctgaacaagcgcggctacggtgtgcgggtcccgaatacgctatcgctgaaggggactcaggaactcatgagcgattggcccattgatgaggtctacaacgtgttggattctaaacaggaagacctcttcgggctgagcgatcttggtcacgaactacctagcggaaggcagcctgagcgtcccatgcgagatagcgacgccagcatcgatgatcaggaaatagctggtgattcgatcggaggcgatcatgttggactgctcccacgggtctggtccatgagccaagacgatccgctgcacaacgtttttgatctgggcggcagtgcgagcggggcgaatggcgcgcagctggcggggccttccccgggtcttggcggcagtaacggttacgctcagggaccaggtggcggaaacggaggctcctctttgatgtacggtgtgagtgcgggcacatttgggaaccaacaaatggcgcttgtttcgagcggcatgggcatgggcagcagcggcgttggtggtggcggcggcggcggcggcggcggctccgaccgcagcatacccgaggtcgtcgtgggagctccaagtagcgtggatgaagattcctacaccgagaaactgcaccgcgtcgattcgtttcatgcactcttgtctgctggtgcaaccacgccacttgcacgcggctcgatcatggagcccactggacgagtcccgggaacaaatcctgactttatgcgcgcgcctccgacggagcatctcagtagcctgagcggcattgtagcgccaaacgccagtcatccgtcgtccgcggtgcatgtgtcgacgtcgggaagccgatcgcttgtgacggctggtggagcggcggcagccctgtcacccggccagatgatgcgcacgcccaacgcggcggttgatccaggtaccacgagcgcatcgccgctgttgctgcaccatactggtggggcgggccacggtcgaggcagttcacgaggcaccgccacgttaccggggtcacagtcgcagccgatgggtactcgatcgatgctgaacgccaacctgcccgggtctgtttttgcgttcgagtccggagaaccgggcgccatgcctcgcccagcaccgggtcattcgctgggacccgaaaccagcgtttccgcacctgcctcgtgggcgcttatcaatgagcgtccgtcgttgtcggcagctgaggatgcgagcgtgcaccggcgacccggcgcgatgccggcatcgacctcgactcggtacgataatggcgaagctgcgcggtatctagaggacagagctggacggaaacgtgcactagctgacgaaggcgtttgcaccaaccctgacttgacgatgccagagaggttccccgcggtggctgccgcgcgagttacgcagcgcttagaacatgatacagcgggcagcgtatcatctgcagcgaaaaccaagcgaagagcgtccggtgctgcagccgcaccgcaagcaccggcccagcagcgaacgcgcgatggatccgccccgaatgaggctcctgctcccggatccagcgccttgcaccatgacgcaacgcgtgcccccgctggaagccgctggctcgagcaaggcgccagtggcgaaagtctcgacgtgcgctcttcgtcggcctcgagcgaccgcacagcaccgatcacccttgagggtctgggagacgtcgagccgccccagacccggagcgaacgactcgaactgctggagcgcatccaccggagcgataacgcgtacgcccgattcgcgggtttccttctccagcactacgatatcacagagaatgtgcgccgaaaccccaagagcacggatttcgtacgtttacggaatctcaaagaccacttcaatcgatacagtgcaccaccacgggctggtcaaggtgccgctcatcgggagccgctcagaatttaccgaatcaaacaatttttcagcaaaatactgaacctggaggtcaccggcgagtgggatcgacacgcacacggcggagtgcgcggcccgtacgtgtacggcctggtgctgcgcgcggatgcgctacagcgtgccgcgccctga

SEQ ID NO: 16 - protein, 1225 aa, Cyanidioschyzon merolae
MSSSRRPSVVWYRGHDLRVEDMPALLAAVQRGGPVVPVFIWAPEEDGMWCLGRPARWWLSRSIVALDRRLRELGCETGLILRRAKSESGGGGGVETTLLEVVKRCGAEAVYWNRVYDPVVLRRDEEVRRRWSKHHRLAVESFKAELLVEPWEVCATESRPASFGDRPLDTFHEFMSAWMAMPPPPEPLPAPKRIEPLIASQSGDQGPLFAVPESTMQPSDVLQSPGGEDTDTEMGIWWNQIHNLGSLEEYWRPGVDCVAERLQDFLTSVFPTYGDARRRQRLRNGTSRLSPYLRFGELSPRRLYHAVRASVLQSEPSDAIIRAARTLLRNLCLREYAYHMLFYRPSILDRPLVPEFDHFPCTKEDVGRLLEVWLSGRTGYPLVDAAMRELHHTGWLHSNLRFLVASFFTKYLLLPWQIRARCLFKLFIDGDLASNAICWQWVTGCNYDVFPLNCLVNPVVMGMRVDPEGEYVRTWCPELQQIPSSYIHAVWKCPPTILHQARVELGVTYPRPVVENRVARRRARDALRYLRQVVLNKRGYGVRVPNTLSLKGTQELMSDWPIDEVYNVLDSKQEDLFGLSDLGHELPSGRQPERPMRDSDASIDDQEIAGDSIGGDHVGLLPRVWSMSQDDPLHNVFDLGGSASGANGAQLAGPSPGLGGSNGYAQGPGGGNGGSSLMYGVSAGTFGNQQMALVSSGMGMGSSGVGGGGGGGGGGSDRSIPEVVVGAPSSVDEDSYTEKLHRVDSFHALLSAGATTPLARGSIMEPTGRVPGTNPDFMRAPPTEHLSSLSGIVAPNASHPSSAVHVSTSGSRSLVTAGGAAAALSPGQMMRTPNAAVDPGTTSASPLLLHHTGGAGHGRGSSRGTATLPGSQSQPMGTRSMLNANLPGSVFAFESGEPGAMPRPAPGHSLGPETSVSAPASWALINERPSLSAAEDASVHRRPGAMPASTSTRYDNGEAARYLEDRAGRKRALADEGVCTNPDLTMPERFPAVAAARVTQRLEHDTAGSVSSAAKTKRRASGAAAAPQAPAQQRTRDGSAPNEAPAPGSSALHHDATRAPAGSRWLEQGASGESLDVRSSSASSDRTAPITLEGLGDVEPPQTRSERLELLERIHRSDNAYARFAGFLLQHYDITENVRRNPKSTDFVRLRNLKDHFNRYSAPPRAGQGAAHREPLRIYRIKQFFSKILNLEVTGEWDRHAHGGVRGPYVYGLVLRADALQRAAP

SEQ ID NO: 17 - DNA, 3147 bp, Cyanidioschyzon merolae
  source 1..3147: mol_type = genomic DNA
atgcccgcgtatcctccttcagaaactagtggagaggagtgtccgtggcttgctttgagcagctccccgttgctcgaagcggggcgggaggtgaacgcgcatccgccaccgggacgtacaccagcgctcgcagtggctgcagcgcagggcgcgacacagcgccccatactggtatggtaccgggggcacgacctccgaatagatgatcatgctgccttctgtgcggctgcagaaacgggtatgccggtggttcctgtgtacgtttggaacccgcaactgccgtggatgagtaaacctggcagagcagggcgctggcggctgcgagagtcgctgctggcgctggaccgggagttcgcgcaccgctacggcgaagatgcgcggctggtggttctgcaggggagcctcgtggaaagcattgtggagctggcgcgggaaacgaatgcgagcgcagtctacttcaaccgctgctacgatatcggtgccgcagaagtggaccgaacgttggaacaacgccttgctgtttggaatgttgaactcgttagcttcaaatcggaacttcttgtggagccgtgggagcttgctcaagacaacggtgagccattcaatgagtttcaccccttcatggaaaagtggctcgctttcccgaaaccgcccccacctgtagcagcgccattgaggctgcagacgctgcctggtttacggcaacgcgtttcccatgtcgagattcatgagctggagctggtctctgatctcagtccggaatggtgtgcccagatggaatgcatgtggccgcttgtcggtgagcgagcagcgtggattacgttgtcaaggtttctccgagagcgttatcccaaattcgggcgtcgagagtctcgttgtgcgctcgacggcacgagccgcctctccatgcatgttcgtttcggtgagattagcccgcggcagctgtatgcagcaatcatggctgacatcgtgtcggacgcgcctagcgcgctttccctagggaatggaataccagcgcattcgagggagcagaacggttacctggagtcgccacaccgaatcagtgcaacacctcactccatggatgctactgctattgctactgctactgctgcagttcccggttatcagccgcagcgagcgccgatgtttccgcttcgggttcaagtgaaccgaccacgaggctccagtggcacgacctactttctctacgatcatgaggatgacgacgacgacgataataataataataatggtgatgaagcagatgacaacgacgacggaggtcgtggtggtaccgatcaagcggctccaaggagcacacggcatgcgctcctgaaccgtgagcgtcacgctacagcaggcgaggcgctcgcggcaaacacacgtacccacaccgatgcagcagatgcacaacagaccatcagcgcggtgaaggcgttcctgaaaaacatgtgcctccgagaattcgcgtatcacctgctctttcacaatccacaggccttcgaagagccgctactgcccgaattccgcgcctttccttggcgctggaacgatcagagcatgctcgaggtttggcgaagcggccaaaccgggtatcccatcattgacgcagcgattcgggagttgcgtaccactggatacctgcataatcgcattcgtttcatgatcgccggcttcctgaccaagtaccttctcattccgtggcagcatcgcctccgctttctttacgatcatgttctcgacggggacatagcctgtcagacgctcgggtggcagtggacggcaggctgccacaccgatgcgttcccgtttgcgtgtatcgtcaatccgatcacgtttgggctcagagaagatccccatggtgagtacgtgaagcgctgggtacccgaattggccgcactgcctacgtgttacgtccatcgtccgtggcgagcgccagcttcagtgcttgcgcaagcgggtatcgcgctgggctcttgctatgcgcatccggtggtggactcgcggacggctcgagcgcgagcactcgactccatggacctcatgcggcgtgtatttgtactgcgacaaccaacccgatccctgtggtctttaattgatctgcaacagccgcagttgtggcttgagcaatctgcatcggattcggacgattccgggatggaaacgttctctttcacgaatggaacgccatacgcacttcatgatcgcttttcaaggggctcaacgaccatcattgaggagctcgccccgaccgtcgagcacaacgctcttcagtcgctttcctatggtaaccacagtcgtcgagcattcggcattggcagtgtacatacagcagcagcgttggtgccagaaagccgacaacgacaacgacgaggctacgcgccctcctggatcgaacgtgcggacgcaggagcgtctgaagttggtgcgatgcagcctggcggacgctcttcggggtcgtcttcgcaactgagtgtagtgcgtcccgagcaactcaatgagtttctccgctgggtaactggtccagaggatgctgccgccaaccaggaacaagcatcggcaacggcaaacgagcagttgcgagcatggaatgacccgctggagcgtgtccagactgcggacattggtcgggagctctcgcctatcacgacgagtgcgcagagcgtgaccctggaaccagcgcagccacagaaacggcgacgtggaggccagcgcaatcctacgcgagcgagcatgctcggtgtagcggaacgcgaagagatattggcagcgatagcgctgcaacctaaccaaccgtttcactgcttcgcgcgcttcctgatgcagcactatcgtttcacaccgaatacggttttcggaccacatacggactttgttcgcttgcgcgcgctcaaagcagagttagctgctgcaggaacatcttgcgaggattcgacgacctccgaaaggagccgctcgtatgaacgacagaaaagccgttgcctcggtcacgttttaactgttgcgaaaatgaagcactttctgcggaatacgcttggactagaggtcactggccagtgggatcgtcgagcgcacggcggggtgcgaggtccgtacgcctacggcctcacgcgctgcccagcgagcgacgacaagcgcagatga

SEQ ID NO: 18 - protein, 1048 aa, Cyanidioschyzon merolae
MPAYPPSETSGEECPWLALSSSPLLEAGREVNAHPPPGRTPALAVAAAQGATQRPILVWYRGHDLRIDDHAAFCAAAETGMPVVPVYVWNPQLPWMSKPGRAGRWRLRESLLALDREFAHRYGEDARLVVLQGSLVESIVELARETNASAVYFNRCYDIGAAEVDRTLEQRLAVWNVELVSFKSELLVEPWELAQDNGEPFNEFHPFMEKWLAFPKPPPPVAAPLRLQTLPGLRQRVSHVEIHELELVSDLSPEWCAQMECMWPLVGERAAWITLSRFLRERYPKFGRRESRCALDGTSRLSMHVRFGEISPRQLYAAIMADIVSDAPSALSLGNGIPAHSREQNGYLESPHRISATPHSMDATAIATATAAVPGYQPQRAPMFPLRVQVNRPRGSSGTTYFLYDHEDDDDDDNNNNNGDEADDNDDGGRGGTDQAAPRSTRHALLNRERHATAGEALAANTRTHTDAADAQQTISAVKAFLKNMCLREFAYHLLFHNPQAFEEPLLPEFRAFPWRWNDQSMLEVWRSGQTGYPIIDAAIRELRTTGYLHNRIRFMIAGFLTKYLLIPWQHRLRFLYDHVLDGDIACQTLGWQWTAGCHTDAFPFACIVNPITFGLREDPHGEYVKRWVPELAALPTCYVHRPWRAPASVLAQAGIALGSCYAHPVVDSRTARARALDSMDLMRRVFVLRQPTRSLWSLIDLQQPQLWLEQSASDSDDSGMETFSFTNGTPYALHDRFSRGSTTIIEELAPTVEHNALQSLSYGNHSRRAFGIGSVHTAAALVPESRQRQRRGYAPSWIERADAGASEVGAMQPGGRSSGSSSQLSVVRPEQLNEFLRWVTGPEDAAANQEQASATANEQLRAWNDPLERVQTADIGRELSPITTSAQSVTLEPAQPQKRRRGGQRNPTRASMLGVAEREEILAAIALQPNQPFHCFARFLMQHYRFTPNTVFGPHTDFVRLRALKAELAAAGTSCEDSTTSERSRSYERQKSRCLGHVLTVAKMKHFLRNTLGLEVTGQWDRRAHGGVRGPYAYGLTRCPASDDKRR

SEQ ID NO: 19 - DNA, 32 bp, synthetic construct
  source 1..32: mol_type = other DNA
gttccagattacgctatgtcgtcgtcgagacg

SEQ ID NO: 20 - DNA, 29 bp, synthetic construct
  source 1..29: mol_type = other DNA
taaatagctagtttatcagggcgcggcac

SEQ ID NO: 21 - DNA, 31 bp, synthetic construct
  source 1..31: mol_type = other DNA
gttccagattacgctatgcccgcgtatcctc

SEQ ID NO: 22 - DNA, 32 bp, synthetic construct
  source 1..32: mol_type = other DNA
aaatagctagtttatcatctgcgcttgtcgtc

SEQ ID NO: 23 - DNA, 19 bp, synthetic construct
  source 1..19: mol_type = other DNA
ggcagatccgcgctcgttg

SEQ ID NO: 24 - DNA, 21 bp, synthetic construct
  source 1..21: mol_type = other DNA
acggcaggagaaggtacttgg

SEQ ID NO: 25 - DNA, 24 bp, synthetic construct
  source 1..24: mol_type = other DNA
gcctccgctttctttacgatcatg

SEQ ID NO: 26 - DNA, 21 bp, synthetic construct
  source 1..21: mol_type = other DNA
atgctgccacggaatgagaag

SEQ ID NO: 27 - DNA, 24 bp, synthetic construct
  source 1..24: mol_type = other DNA
cgccagggttttcccagtcacgac

SEQ ID NO: 28 - DNA, 24 bp, synthetic construct
  source 1..24: mol_type = other DNA
gagcggataacaatttcacacagg

SEQ ID NO: 29 - DNA, 23 bp, synthetic construct
  source 1..23: mol_type = other DNA
tctgctcggcttagtttcgaaag

SEQ ID NO: 30 - DNA, 23 bp, synthetic construct
  source 1..23: mol_type = other DNA
taccccgattcgatcatacgagt

SEQ ID NO: 31 - DNA, 2046 bp, Arabidopsis thaliana
  source 1..2046: mol_type = genomic DNA
atgtctggttctgtatctggttgtggttctggtggttgtagtattgtatggtttagaagagatcttagggttgaagataatccagctttagcagcagcagtaagagctggtccagtgattgctctgtttgtttgggcaccagaagaagaaggacactatcatccaggtagggtttctaggtggtggctcaagaacagtttggctcagcttgattcttctcttagaagtcttggtacttgtcttatcaccaagagatctactgatagtgttgcttctcttcttgatgttgttaaatccactggtgcttctcagatcttcttcaaccatttgtatgatccattgtctttggtgcgtgatcaccgagctaaagatgttttgacggcgcaaggcatagcggttcgatcattcaacgcagacttgctttatgagccatgggaagtgactgatgaattaggccgtcctttctctatgtttgctgcgttttgggagagatgtcttagtatgccttatgaccctgagtctcctcttcttccacctaagaagatcatttcaggggatgtgtctaaatgtgttgcggatccattggtgtttgaggatgactctgagaaaggaagcaatgcacttctggctcgtgcttggtctcctggatggagtaatggtgataaagctctcacaacgtttataaacggtccattgcttgaatactctaagaaccgcagaaaagccgatagtgctacaacctcgtttctttctccacacttgcattttggggaagtgagtgtgagaaaagtttttcatcttgttcggatcaaacaggtcgcgtgggcaaacgaaggaaacgaggccggggaagaaagcgtgaatcttttcctgaaatctattggtctcagggagtattctaggtacataagttttaaccatccatattcccatgaaagaccacttcttggccatctaaagttcttcccttgggctgtggatgagaactatttcaaggcatggaggcaaggccggactggatatccgttggtcgatgccgggatgagagagttatgggctactggttggttgcatgatcgcataagagtagttgtttcaagcttctttgttaaagtgcttcaattaccatggagatgggggatgaagtatttctgggacacacttcttgatgcggatttagaaagcgatgctcttggttggcaatacattaccggtactctcccggatagccgggagtttgatcgcatagataaccctcagtttgaagggtacaagtttgatccaaatggtgaatacgtaaggcgatggcttcctgaactctctagactcccgacagactggatacatcatccgtggaacgcacctgagtccgttcttcaagctgctggtatcgagcttggatcaaactatcctctaccaattgttggattagacgaagcaaaagcacggcttcatgaagcgctttcacagatgtggcaactagaagctgcttcaagagctgcaatagagaacggatccgaagaaggacttggagattctgctgaggtagaggaagctcctatagagttcccaagggacattacaatggaagagactgaaccaaccagactcaacccaaacaggagatatgaggatcagatggttccaagcattacttcttctttgatcagacctgaagaagacgaagagtcgtctcttaatttgagaaattcagtaggagatagcagagcagaggttccaaggaacatggttaacaccaaccaagctcagcagcggagagcagaaccggcttcaaaccaagtcactgctatgattccagaatttaatatcagaattgttgcagagagcactgaagactcaacagcggaatcttccagcagcggaaggagagaaagaagcggaggcatagtccccgagtggtctccagggtactcagagcagttccctagtgaagaaaatcgtattggaggaggaagtacaacgtctagctacttgcagaatcaccatgaaatactgaactggagacggctttcacaaaccgggtaa

SEQ ID NO: 32 - protein, 681 aa, Arabidopsis thaliana
MSGSVSGCGSGGCSIVWFRRDLRVEDNPALAAAVRAGPVIALFVWAPEEEGHYHPGRVSRWWLKNSLAQLDSSLRSLGTCLITKRSTDSVASLLDVVKSTGASQIFFNHLYDPLSLVRDHRAKDVLTAQGIAVRSFNADLLYEPWEVTDELGRPFSMFAAFWERCLSMPYDPESPLLPPKKIISGDVSKCVADPLVFEDDSEKGSNALLARAWSPGWSNGDKALTTFINGPLLEYSKNRRKADSATTSFLSPHLHFGEVSVRKVFHLVRIKQVAWANEGNEAGEESVNLFLKSIGLREYSRYISFNHPYSHERPLLGHLKFFPWAVDENYFKAWRQGRTGYPLVDAGMRELWATGWLHDRIRVVVSSFFVKVLQLPWRWGMKYFWDTLLDADLESDALGWQYITGTLPDSREFDRIDNPQFEGYKFDPNGEYVRRWLPELSRLPTDWIHHPWNAPESVLQAAGIELGSNYPLPIVGLDEAKARLHEALSQMWQLEAASRAAIENGSEEGLGDSAEVEEAPIEFPRDITMEETEPTRLNPNRRYEDQMVPSITSSLIRPEEDEESSLNLRNSVGDSRAEVPRNMVNTNQAQQRRAEPASNQVTAMIPEFNIRIVAESTEDSTAESSSSGRRERSGGIVPEWSPGYSEQFPSEENGIGGGSTTSSYLQNHHEILNWRRLSQTG

SEQ ID NO: 33 - DNA, 2988 bp, Haematococcus lacustris
  source 1..2988: mol_type = genomic DNA
atggaccgctcggcgcctgtaatttggtggtgccgtagagacttacgagtggatgacaacccttcgcttctcgcagcgttgcaaagctcaccaaacctgatccccgtgttcatttgggctcccgaggaggagggacagttccagcctggccgcttcagccgttggtggacaaaacagtccgtcgctctgttccagcgactgctgggtcggctaggctcccggctcattattaggcggtgttcggacacagctcaatgcatcacccaagtagtagcagagacgggcgccaaggcagtgtattttaaccatctgtacgacccaatttcgctggtgcgagaccatgaggtgaagacagctctggcgaagttaggcgtggagtgtcgcagcttcaattcggacctgctctacgagccctgggagttgctggactcagctggcgagccctttacaagttttgagacgttttggaataggaccttggcaatgccctaccccccacccttccctttgcctgcgcctcaccagcttccaccagtcagccctaacatagacagtacaccactggagaaggtggactggttccagacacctgaacaggaggcttcttgtgaccagctgcgcttcaagtggaagcctggtgtggagggtgctgtggagaagctcgagtcattcttgaccaataggctcacatcgtttgaggcagatcgggcaaaagttgaccgtgacagcaccagccaactgtcgccatggattcacattggcaccatcagtgtgcgctacattttctatcgggtttgccagcagcaggctgaatgggctgcagcagcatctagcccactggtgcccccccaggccctgccctccatcacgaacagttgcaaagactttctgcagcagatgggctaccgcgagtattcccgctacctgtccttccatttccccttcatcacagaaagggcgttactggcccacctgcgagcctgcccctggcgcctggaccaagccgccttcaaggcatggcgtcagggacagactgggtaccccttagtggacgcggccatgcgtcaattgtccagcaccggctggtgccacaaccgcatgcgagtcgtggctgcgtcgttcatggtgaaaaacctgctcttaccatggcaatggggcttgaagcactattgggatgcccagctggatgctgacctggagtgtgatgccctgggttggcagtatgtgtcgggcggcatggcagatgctcacccttttaaccacatcattgacctggagaaggaggcgcagcggtttgatgctgatggggagtatgtgaggcgctggctgccagtgctgtcccgcatgcccacccagcatatccacgccccctggcgagctccccatgctgtgttggcggcagctgatgtggagctgggttttgactaccctgaacgggtggtcactgctgaggagtctgcacgcaacatggctgaggcttgtcacgtgcttcagcactgccaggccagtggcagcagtgaccgacggtctggcccctaccgcaccgccaccttagacctggccctggcagtggctgctggtgtggctcggggcagcagtggcgctggcactggcactggctttgtcctgtgtggcgagcaagggagtgcaggcaacaagggcagcaacgagcaggacatggcaggctccgtcccagcgctgctccaggaggcccctccacttgtcattgccagcctgcagcagaggcgaagcagtgcaggcccagggcagcagcagctgttgggagcaagagctgggacggtcagaatcggggcaggggctggggcagggtcaaaggctgcactgcccactgcagaacaggcagtgcatgatgccgccgtcaaggcagctgatgtggtggcaggggatcgctggctgggtggcccgccccagcctgcatacccgggcactgacttccgcaaaccaggcatgcagggcaatgacggcagagaagggaggggtgagggccaggggcatggagcatggcgccggcgtatggggcgtgcttgccagcaacacagcaccccattctgccagcccatggcttctgagggggcctcccggcatgctgctcctgcacattatgaggttcctgctggccgttaccaccaccaccaccagcaccgccaccagcggcaggcacaagggcaggaggagggtgaaggccagagagaacagggctgtggtggacctggcaggtccgggctggcagactttgcaagggagctgttggtcatggagccagcaggggctccagggcagcctggagtgcagcctacgccagcgtcctggcaggatggccagcatgaagggggccccttcaactctggctacatctccaccagctcaggctgctcagaggacatggaggcgatgtcagaggaggtggtcagcaacaccataggcctctcccgcacccagacctccggctggagctgccccagaccccaggcccctgcgcccttccctcagaccgcaggtcttggtggacccgctgcagcacgtgctgctgccatggcggctgagggcccatcggtctgcaccctgccagtctcaggtccaggatcagggcggaggccatctggtactatgggtgctgctgccagctctgtggcagacaatgatggccatggggcagtatctgcggcgccgacaaaccctgagcagcaatggtgcacacctgttgggtcagccgctgcccctgagcctgaaggtgggcaggacgtggacatggttggcagcagggacaccagccccgacacctccctggaccagcagcaggaccagcacggcctgcagcagcaggcgtcacagccgccactgcagcagcaatggcacacgcctgcgcagcatctgctgcactatgctacatcccagccttcagtatccccatcccggccccataccaaaacctcctcacttgcactagctgctgtgcattgcccctaa

SEQ ID NO: 34 - protein, 995 aa, Haematococcus lacustris
MDRSAPVIWWCRRDLRVDDNPSLLAALQSSPNLIPVFIWAPEEEGQFQPGRFSRWWTKQSVALFQRLLGRLGSRLIIRRCSDTAQCITQVVAETGAKAVYFNHLYDPISLVRDHEVKTALAKLGVECRSFNSDLLYEPWELLDSAGEPFTSFETFWNRTLAMPYPPPFPLPAPHQLPPVSPNIDSTPLEKVDWFQTPEQEASCDQLRFKWKPGVEGAVEKLESFLTNRLTSFEADRAKVDRDSTSQLSPWIHIGTISVRYIFYRVCQQQAEWAAAASSPLVPPQALPSITNSCKDFLQQMGYREYSRYLSFHFPFITERALLAHLRACPWRLDQAAFKAWRQGQTGYPLVDAAMRQLSSTGWCHNRMRVVAASFMVKNLLLPWQWGLKHYWDAQLDADLECDALGWQYVSGGMADAHPFNHIIDLEKEAQRFDADGEYVRRWLPVLSRMPTQHIHAPWRAPHAVLAAADVELGFDYPERVVTAEESARNMAEACHVLQHCQASGSSDRRSGPYRTATLDLALAVAAGVARGSSGAGTGTGFVLCGEQGSAGNKGSNEQDMAGSVPALLQEAPPLVIASLQQRRSSAGPGQQQLLGARAGTVRIGAGAGAGSKAALPTAEQAVHDAAVKAADVVAGDRWLGGPPQPAYPGTDFRKPGMQGNDGREGRGEGQGHGAWRRRMGRACQQHSTPFCQPMASEGASRHAAPAHYEVPAGRYHHHHQHRHQRQAQGQEEGEGQREQGCGGPGRSGLADFARELLVMEPAGAPGQPGVQPTPASWQDGQHEGGPFNSGYISTSSGCSEDMEAMSEEVVSNTIGLSRTQTSGWSCPRPQAPAPFPQTAGLGGPAAARAAAMAAEGPSVCTLPVSGPGSGRRPSGTMGAAASSVADNDGHGAVSAAPTNPEQQWCTPVGSAAAPEPEGGQDVDMVGSRDTSPDTSLDQQQDQHGLQQQASQPPLQQQWHTPAQHLLHYATSQPSVSPSRPHTKTSSLALAAVHCP

SEQ ID NO: 35 - protein, 12 aa, Haematococcus lacustris
LLLPWQWGLKHY

SEQ ID NO: 36 - DNA, 1776 bp, Nannochloropsis gaditana
  source 1..1776: mol_type = genomic DNA
atgccctggaaattcctattgaccctcgcactagctatctccctatcactggcgtaccttccgcggagtgcttcctttgtccgtcctatcacaatgaccagtacagctgtctccaagcctgctgcgaaaggggcagctcgcacggtttctctccattggttccggaaaggcttgcgtttacacgataatcctgccctgttggaggcatgtgaaggagccacgcatgtgtaccccgtgttcatcctcgatccacacttcgccaagcccgacgtcattggcgtcctgcggtaccgattcatgctgcaaacgatcaagaacctggatgacaatttgcgtgaaatcggttctcggttgttcgtggtcaagggtcaaccggcggaggccctgccccggctttttagggagtggggagtgacgaaactcacgttcgaaagcgacaccgagccctacgccaaggtccgcgaccgacacgtgtgcgagcttgccgcggagcaccaggtgcatgtccagactttcccctcgcacacccttcacgaccccgaggcttacgtggcgcgcctgcaggggaaggatgtgcccacagtctaccagtccttcgtgaagctattcgcctccatgggccccgtggcccccgtggcttcgactgttgacgccaagcggctcccacccccggcgctggagtatttgtcgggtcaagacggaaagaaggctggccaagggaacgggcatgctggaggcgaggagatagaggaagaccggacacgaggcgacgatttctccgtccctggtctctcgggaataggctacccggagacggatgcccctaccctgtatcccgggggggagacggcggccctggcccggatgcaggagcatctggccaatgtcaagtacatcgtcacgttcgagaaacccaagacctctcccaacgccctccggccctccacgaccgtcctctctccttacttgaagcacggggccctgtcctcccgcctcttttaccactccctgcgctccatccttgcgcagcacaagggcccccacacccagcccccggtctccctggtagggcagctgctctggcgcgagttcttctacctgcaggggcacgccacgcccaatttcgacaagatggtggggaacccgatctgccgacagatcccatgggggaagaacgcggagcttctgggcgcctgggaagaggcgcggaccggataccctttcattgacgcgtgcatgacgcagctccgggaggaaggctggatccaccatctggcccggcacgccctggcgtgttttttgacgcggggggacctgtggcagagctgggaggaaggggcgagggtgtttgagaagtacttattggacgccgactggagcgtgaatacagggaactggctctggctctcggcgtcggccttttttcaccagtacttccgggtctattcccccgtggctttcggggccaagacggacaaggagggcgagtacatccgcaagtatctgccggtgctgcggaaaatgccaatcaagtacatttatgaaccttggaaagcccccaaaggtgtccaagaaacagcgggctgtgtggtgggccgagactaccctcacccggtggtcgaccatgccacagtcagcaagcagctgatgggcaagatgaaggcggcttacgacgcaaacaaggagggggggggcaaagggggggagaagtctggcgagaagaagaggccggcgggggaggacggaaaggggggtaagactaagaagcgggcctaa

SEQ ID NO: 37 - protein, 591 aa, Nannochloropsis gaditana
MPWKFLLTLALAISLSLAYLPRSASFVRPITMTSTAVSKPAAKGAARTVSLHWFRKGLRLHDNPALLEACEGATHVYPVFILDPHFAKPDVIGVLRYRFMLQTIKNLDDNLREIGSRLFVVKGQPAEALPRLFREWGVTKLTFESDTEPYAKVRDRHVCELAAEHQVHVQTFPSHTLHDPEAYVARLQGKDVPTVYQSFVKLFASMGPVAPVASTVDAKRLPPPALEYLSGQDGKKAGQGNGHAGGEEIEEDRTRGDDFSVPGLSGIGYPETDAPTLYPGGETAALARMQEHLANVKYIVTFEKPKTSPNALRPSTTVLSPYLKHGALSSRLFYHSLRSILAQHKGPHTQPPVSLVGQLLWREFFYLQGHATPNFDKMVGNPICRQIPWGKNAELLGAWEEARTGYPFIDACMTQLREEGWIHHLARHALACFLTRGDLWQSWEEGARVFEKYLLDADWSVNTGNWLWLSASAFFHQYFRVYSPVAFGAKTDKEGEYIRKYLPVLRKMPIKYIYEPWKAPKGVQETAGCVVGRDYPHPVVDHATVSKQLMGKMKAAYDANKEGGGKGGEKSGEKKRPAGEDGKGGKTKKRA

SEQ ID NO: 38 - protein, 12 aa, Nannochloropsis gaditana
LWQSWEEGARVF

SEQ ID NO: 39 - DNA, 1683 bp, Nannochloropsis gaditana
  source 1..1683: mol_type = genomic DNA
atgaccagtacagctgtctccaagcctggtgcgaaaggggcagctcgcacggtttctctccattggttccggaaaggcttgcgtttacacgataatcctgccctgttggaggcatgtgaaggagccacgcatgtgtaccccgtgttcatcctcgatccacacttcgccaagcccgacgtcattggcgtcctgcggtaccgattcatgctgcaaacgatcaagaacctggatgacaatttgcgtgaaatcggttctcggttgttcgtggtcaagggtcaaccggcggaggccctgccccggctttttagggagtggggagtgagcaaactcacgttcgaaagcgacaccgagccctacgccaaggtccgcgaccgacacgtgtgcgagcttgccgcgaagcaccaggtgcatgtccagactttcccctcgcacacccttcacgaccccgaggcttacgtggcgcgcctgcaggggaaggatgtgcccacagtctaccagtccttcgtgaagctcttcgcctccatgggccccgtggcccccgtggcttcgactgttgacgccaagcggctcccacccccggcgccggagtatttgtcgggtcaagacggaaagaaggctggccaagggaacgggcatgctggaggcgaggagatagaggaagaccggacacgaggcgacgatttctccgtccctgatctctcgggaataggctacccggagacggatgcccctaccctgtatcccgggggggagacggcggccctggcccggatgcaggagcatctggccaatgtcaagtacatcgtcacgttcgagaaacccaagacctctcccaacgccctccggccctccacgaccgtcctctctccttacttgaagcacggggccctgtcctcccgcctcttttaccactccctgcgctccatccttgcgcagcacaagggcccccacacccagcccccagtctccctggtagggcagctgctctggcgcgagttcttctacctgcaggggcacgccacgccaaatttcgacaagatggtggggaacccgatctgccgacagatcccatgggggaagaacgcggagcttctgggcgcctgggaagaggcgcggaccggataccctttcattgacgcgtgcatgacgcagctccgggaggaaggctggatccaccatctggcccggcacgccctggcgtgttttttgactcggggggacctgtggcagagctgggaggaaggggcgagggtgtttgagaagtacttattggacgccgactggagcgtgaatacagggaactggctctggctctcggcgtcggccttttttcaccagtacttccgggtctattcccccgtggctttcggggccaagacggacaaggagggcgagtacatccgcaagtatctgccggtgctgcggaaaatgccaatcaagtacatttatgaaccttggaaagcccccaaaggtgtccaagaaacagcgggctgtgtggtgggccgagactaccctcacccggtggtcgaccatgccactgtcagcaagcagctgatgggcaagatgaaggcggcttacgacgcaaacaaggagggggggggcaaagggggggagaagtctggcgagaagaagaggccggcgggggaggacggaaaggggggtaagactaagaagcgggcctaa

SEQ ID NO: 40 - protein, 560 aa, Nannochloropsis gaditana
MTSTAVSKPGAKGAARTVSLHWFRKGLRLHDNPALLEACEGATHVYPVFILDPHFAKPDVIGVLRYRFMLQTIKNLDDNLREIGSRLFVVKGQPAEALPRLFREWGVSKLTFESDTEPYAKVRDRHVCELAAKHQVHVQTFPSHTLHDPEAYVARLQGKDVPTVYQSFVKLFASMGPVAPVASTVDAKRLPPPAPEYLSGQDGKKAGQGNGHAGGEEIEEDRTRGDDFSVPDLSGIGYPETDAPTLYPGGETAALARMQEHLANVKYIVTFEKPKTSPNALRPSTTVLSPYLKHGALSSRLFYHSLRSILAQHKGPHTQPPVSLVGQLLWREFFYLQGHATPNFDKMVGNPICRQIPWGKNAELLGAWEEARTGYPFIDACMTQLREEGWIHHLARHALACFLTRGDLWQSWEEGARVFEKYLLDADWSVNTGNWLWLSASAFFHQYFRVYSPVAFGAKTDKEGEYIRKYLPVLRKMPIKYIYEPWKAPKGVQETAGCVVGRDYPHPVVDHATVSKQLMGKMKAAYDANKEGGGKGGEKSGEKKRPAGEDGKGGKTKKRA

SEQ ID NO: 41 - protein, 12 aa, Nannochloropsis gaditana
LWQSWEEGARVF

SEQ ID NO: 42 - DNA, 1755 bp, Phaeodactylum tricornutum
  source 1..1755: mol_type = genomic DNA
atgtcgaatagcgaccatggtggcaaacagcggatccttgcaccagcggtccaagcgcattccttatcaaggccagctgtcgttctctttggaactcatgacatccgaattcacgataacgaggccttgctgttggcctgccatcacaaccacgtattgccggtttttctatggcaagtaccggtccaccattggggagctcgtggcgccctgcaagtcgtgttgaaagaagcattgcaccagctttcactacagctttcacaagaaagtatcaatctacctctggtgtgcggcaatacggcggacagtgtttcggagctctgtaaaattgcttctgagattggcgcgagtgcagtctattggaatcgcgagatgacacctgaaagcagggaaatggagaggcacagagccacaagtttgaagcaactcgatatcgcagctgtagcatgtcaatcggccctactctacgatgtcgagaaacttgaacttgacgaggggtttcatggtggtcactggggcacgctgatgccgtttaagagggcttgcgaaaagcaacttggaaaaccggatcgaccgattttgatgaaagagtcgctggcttgcctatactccgtcgctccgcctccgcaagactgtaaatccgtacccatcgaggaactcggcttcgagaccgtgccgccttccacaaagtgggatgagcccattcgagagcgattcccaatgatacattacttggctcagcggagactggaccactttcttataaaagggctacctctgtatgaaagtgaccgaagtcgggcagacatggaatacgcgacttcgcagctttcagtgtaccttcgtattggtatcatatcaccacgagagctatactggaggattgaggacagctcactgagccctgaggcgaagaaaacgtttgcccgtcgactaatctggcgtgagctggcgtactatcaactattctgttttccaaagatgagggacagatcgatacgcaagcactatgaagcatcggaatgggtcacgggtgacgaagagaaaggcagattcaatgcatggaagagagggttgactggctatccgttggtggatgctgggatgcgtgaactctatacaactggttacttgacccaatccgtgcggatggttgtcgcgtcatttcttgtcgagtatcttcgagtcgactggaccaaaggagcagaatggttccactacactttggccgacgccgatagcgcgatcaattcgatgatgtggcagaacgctgggcggagcggcatcgaccagtggaattttgttttgagtcctgagaatgcatcccaagacccatacggagaatatactcgcaaatgggtccccgagctttctccgttgccattgcaatacttacagcgaccttggcagacgtttgaaggtgatcttcgtatggccggtatcgtccttggtgaaacatacccacatagaattgttcaggacctcaagggtgaacgacaaaaaagtgtcgagagcgttcttgcaatgagaaggcgatcgcaagaaaaaaatgatgaaaatggatacgacttgatcgaccttccttcgggcatcgaaacggtcgtttttacgaagaaagagtaccgtattgatcggttgggcaaagtgctccagggaaaaccaaagaccgctacttcaacagtcaagcgccgaaaaacaaaacgtacaacgaaaacagatgggagaagaaagaaccggctgccatcaagtctcgca

SEQ ID NO: 43 - protein, 585 aa, Phaeodactylum tricornutum
MSNSDHGGKQRILAPAVQAHSLSRPAVVLFGTHDIRIHDNEALLLACHHNHVLPVFLWQVPVHHWGARGALQVVLKEALHQLSLQLSQESINLPLVCGNTADSVSELCKIASEIGASAVYWNREMTPESREMERHRATSLKQLDIAAVACQSALLYDVEKLELDEGFHGGHWGTLMPFKRACEKQLGKPDRPILMKESLACLYSVAPPPQDCKSVPIEELGFETVPPSTKWDEPIRERFPMIHYLAQRRLDHFLIKGLPLYESDRSRADMEYATSQLSVYLRIGIISPRELYWRIEDSSLSPEAKKTFARRLIWRELAYYQLFCFPKMRDRSIRKHYEASEWVTGDEEKGRFNAWKRGLTGYPLVDAGMRELYTTGYLTQSVRMVVASFLVEYLRVDWTKGAEWFHYTLADADSAINSMMWQNAGRSGIDQWNFVLSPENASQDPYGEYTRKWVPELSPLPLQYLQRPWQTFEGDLRMAGIVLGETYPHRIVQDLKGERQKSVESVLAMRRRSQEKNDENGYDLIDLPSGIETVVFTKKEYRIDRLGKVLQGKPKTATSTVKRRKTKRTTKTDGRRKNRLPSSLA

SEQ ID NO: 44 - protein, 12 aa, Phaeodactylum tricornutum
LRVDWTKGAEWF

SEQ ID NO: 45 - DNA, 1653 bp, Phaeodactylum tricornutum
  source 1..1653: mol_type = genomic DNA
atggctaaatcggaagagaaaaaacacgacgttgccatccattggttccgcaatggtctccgcttccacgacaacccttgtttgctggatgcgtgccaaaaatccgaatcactccttccgatttacgtagtcgaccctgaatttcccttcgcgcaaactgctgggtgccgcgccggtacaattcgtgccaatttcttactcgaatcgataaacgaagtcgacgaaaaactccggaaaatgggtagtcagctcgtcgttgttctcgggaagagtcacgaagtcttacccgaaattgtcgccaccacacaggctaaggcattgttctatgaacaagaagcagccgctcctgtgcgagagcaagacgccgagacgatccaagccatcaagaatcgtttgaaaagggacggtaaaaattacgagtgcaaatttgaagcctatgcaacgcatacgcttcatcccatggaacggtatttagcgcagtgcaaagaccatacggcaccgtcgacgtatggaagttttacgaagattttcaacaaaatgagtgttgcgaaagaagtgaacgaagtcaaggaggtaccatcgttgccaaacaagtcagttaaacttcttgaaaaatcgtttgcagaggctttgcgaatgcctacgttaaaagatcttggatacgcagctgctgctgatgatatgaagaacagcggcaaaggagggtatgcttttgcagggggagaaaacgccgcaatcgagcttcttgcaaagaacatggcgcgctcgcagtgggtagcaacgtttgaaaaaccaaagacaagcccaaatgatgccacacgaccaagcactactgctttgagtccttacgtcaagcacggctgtatatctccgcgtcgcttttatcatgagttgtcgaaggtgtactcaaaatacaatagcaaagaaacatcgaagccaccagtttcgctccatggacaactaatgtggcgcgacttcaattatctggtcggatacagcactccaaactttgacaaaatgatcgacaatcctattgctcgacaaattccatgggacgacgatccggatcttttgctagcctggaagatgtcgaagacgggatatccttacatcgatgcgatcatgacccaactacgggaaacgggctggattcaccacctagctcgtcattccgttgcttgcttcctcactcgaggggatctatggcaaagctgggaagatggcgctacagtcttcgaagaatatttgattgacgctgattggagcatcaacaacttcaactggcaatggctttcttgcactgcccatttctatcagtattttcgatgctattcgccaattgctttcggtaaaaagacggacccaaatggcgattacattcgcaaatggttgcctcagttcaaggacatgccagcaaagtatatctacgaaccttgggaagctcccattgaacttcaaaagaaagttggggtgattgtcggtgaaaactaccctcatccaattgttgaccacaagttggtcagtaaaaacaatatgtcacggatgaaggaagcgtacgatgcacagaagaatcgggagcctatgccagccaacgaatcgcatagtagcggtttgaatcgtgatacttcaccaaagcgacaacgtcgcaactaa

SEQ ID NO: 46 - protein, 550 aa, Phaeodactylum tricornutum
MAKSEEKKHDVAIHWFRNGLRFHDNPCLLDACQKSESLLPIYVVDPEFPFAQTAGCRAGTIRANFLLESINEVDEKLRKMGSQLVVVLGKSHEVLPEIVATTQAKALFYEQEAAAPVREQDAETIQAIKNRLKRDGKNYECKFEAYATHTLHPMERYLAQCKDHTAPSTYGSFTKIFNKMSVAKEVNEVKEVPSLPNKSVKLLEKSFAEALRMPTLKDLGYAAAADDMKNSGKGGYAFAGGENAAIELLAKNMARSQWVATFEKPKTSPNDATRPSTTALSPYVKHGCISPRRFYHELSKVYSKYNSKETSKPPVSLHGQLMWRDFNYLVGYSTPNFDKMIDNPIARQIPWDDDPDLLLAWKMSKTGYPYIDAIMTQLRETGWIHHLARHSVACFLTRGDLWQSWEDGATVFEEYLIDADWSINNFNWQWLSCTAHFYQYFRCYSPIAFGKKTDPNGDYIRKWLPQFKDMPAKYIYEPWEAPIELQKKVGVIVGENYPHPIVDHKLVSKNNMSRMKEAYDAQKNREPMPANESHSSGLNRDTSPKRQRRN

SEQ ID NO: 47 - protein, 12 aa, Phaeodactylum tricornutum
LWQSWEDGATVF

SEQ ID NO: 48 - DNA, 1956 bp, Diacronema lutheri
  source 1..1956: mol_type = genomic DNA
atggtggcggaggatgcgcagccggtgctggtgtggttccggcgcgacctgcggctggccgaccaccgcgcgctgcacgcggcggctggatcgggcgcgcccgtcgtgcccgtgtacgtgcacgcgccggacgaggaggggccgtggccgctcgggggcgccgcgcgccgctggctgctgcgctcgctcggcgcgctgcgcgacgagttgcgctcgcggctgcgctcagagctcgtgcttcgcgtagcggagcgtggcgttggctcggcatcagcgctcgtagcgctcgccatcgaggtgcgcgcgagcgcgtgctacttccaccgcgagtacgagccgtggagcctcgagcgcgacgacgcggtgcgcgcggcgctcggcgcggtcggcgtcgagagccgcaccttcgtcggcggtgtgctcaacgagccgtgggccgtgcgaccggacgagcgcccgcgcgccgtggccgtcggcttcggcacgtacgccatgtgggcggccgccgtcgacgaggcgaacgacgaggcgcgcgcggccgctccggcgggcatggcgcttgaaccggcggaagagccgctccccgcaccgagcgcgctgcccgcgccgccggcgggctttccggcctccgtgccgctcgccagctttgcgctcgcaccggcgccgccgagcgcaaccgccgcgcccgcgggcgacgacgacgccgactcttccgacgggcgcgacgcgcgtcgggctggcattgccggtggcacgtgggccgtcggcgaggccgccgcgctcgccgcgctcgctgccttcgtcgccgacggcctcggctggtacgcgagccgcgagcgcaaccgcgctgaccgaccgtgcagcacctcgcgcctctcgccgcacgtacgcgcgggcgagctgagcccccgacagctgctcgcggccgcacgcggggccggcgacgacgcggcggcgggcgcgctctaccgccgcctcgcgtggcgcgacatggcgtactgggcgctgtggcgcttcccgccgccgcgcgccgcgctgctgcgccgcgccggcgcgcgcgacggccaagccacggcggagggcgacacgggcacgcgtacacttggctggctcgagggcttccggccacagtatggcgcggaggcgtgggcggacgacggtggcgaattgctgagcgcgtggcagctcgggcgcaccggctacccgctcgtcgacgcggcgatgcgcgagctgcgtcgaacggggtggatggccaactacttgcggcatgtgtgcgcccagttcctcgtcgagtacctgctcgtcgactggcggcatggcgcgcgctggttcgcgagtgcgctcgtcgacgcggacacggcggtcaatctcttcatgtggcagaacggagggcactgcggcctcgaccagtggtgcttcgtgatgcacccggtgcgtgcggcggcatcgtgcgacccagaaggcctatacgtgcgtgcacaattgcctgagctcgcgcgcctgccggccgagtacgcgcatcgcccgtgggacgcgcccgacgacgtgctcgcgcgcgcgggcgttgcgctcgggcccggcggcacgtacccgcgccgcatcgtcgtcgaccttgacgcagcgcgcgcgcgcacgcacgacgccgtgctgcgcgcgcgcgcgcgcacctacggcaggctcgtcggcgcgggcggcgtcgacgttctcgagctcgacgggcagcggcacgcgctcgtcacgcgcaaggagctccgagcgacggggagcgccgcgcgcgtcggagcgcgcgcctccgacgcgcgcggcggcgcaggcgcggcctcggacggcgcgagcgcgcagaccggacgcgcggctcgagcaccgcgccagcgcgcgcgcgcgcgatccgagacagccgcgacggacgcagctgcgggcagtgcccgtgcgccggccgtgcgcgatggcgtctga

SEQ ID NO: 49 - protein, 651 aa, Diacronema lutheri
MVAEDAQPVLVWFRRDLRLADHRALHAAAGSGAPVVPVYVHAPDEEGPWPLGGAARRWLLRSLGALRDELRSRLRSELVLRVAERGVGSASALVALAIEVRASACYFHREYEPWSLERDDAVRAALGAVGVESRTFVGGVLNEPWAVRPDERPRAVAVGFGTYAMWAAAVDEANDEARAAAPAGMALEPAEEPLPAPSALPAPPAGFPASVPLASFALAPAPPSATAAPAGDDDADSSDGRDARRAGIAGGTWAVGEAAALAALAAFVADGLGWYASRERNRADRPCSTSRLSPHVRAGELSPRQLLAAARGAGDDAAAGALYRRLAWRDMAYWALWRFPPPRAALLRRAGARDGQATAEGDTGTRTLGWLEGFRPQYGAEAWADDGGELLSAWQLGRTGYPLVDAAMRELRRTGWMANYLRHVCAQFLVEYLLVDWRHGARWFASALVDADTAVNLFMWQNGGHCGLDQWCFVMHPVRAAASCDPEGLYVRAQLPELARLPAEYAHRPWDAPDDVLARAGVALGPGGTYPRRIVVDLDAARARTHDAVLRARARTYGRLVGAGGVDVLELDGQRHALVTRKELRATGSAARVGARASDARGGAGAASDGASAQTGRAARAPRQRARARSETAATDAAAGSARAPAVRDGV

SEQ ID NO: 50 - protein, 12 aa, Diacronema lutheri
LLVDWRHGARWF

SEQ ID NO: 51 - DNA, 1746 bp, Diacronema lutheri
  source 1..1746: mol_type = genomic DNA
atggccgggtcgacgaagacggccaggggcgcgatggttgtgctgctgtggtaccgcaaggggctgcgcgtgcacgatagcccggcgctcgccgcggcgtgcgagggcgcgaccgccgtgtgccccgtcttttgcctggacccgtggttcgtctcgtcgggcaaggttgggccaatccgcctccgcttcctcgccgaggcgctcgccgacctcgacgcgtcgctgcgcgcgcgcggctcgcggctgcttgtgctgcacggcaagcctgaggaggagctaccgcgggttgcgcgcgagtggggcgccacacatatcgtctgggagaaggacggcgtggagccatacggcctcaagcgcgacgcggccgtgcgcgaggcgtgtgcgccgctcggcgtgacgatcaccgagacgaacggtcacacgatctgcgacctcgacgagctgctcaagcagtccaagggctcgccggtgacgacgtattcgacattccgcacgcactttgaccacgtcgtcgcgcgctcgcccatcgtgctcacgcccacgcccgagcggatcccggcgccgagcgacgctgcgctggccgaggaggcgcgcggccgcctctccgttccgtccgtcgcggacatcgcgccgtcgctcgcggacgcgggcccgtcgctcttccccggcggcgagggcgaggcgctgcgccggctcgacgcgcacctcgcgcgcgatggcggcgcgtgggccggcgcgtttgaaaagccaaagacgagtccaaccgaaattgaccccttcggagccggcacgcgctcgacgacggtgttgagcgcctacctcaagttcggctgcctctcgccgcgcaccttttgggtgcgcttgcgcgacgcgaccaagggcgcgcgcacccgctccgcgccgcccgtctcgcttgacggccagctcctttggcgcgagttttattacgcatgcgcgcacgccgtcggccctgcgtttggacaaatggaggacaacccgatttgccggcagatcggctggcgcgtgccggcggacgatccagcggcggccgaggcgctcgccgcgtggcgcgacgggcgcaccggctacccatggatcgacgcatgcatgcgccaactgaagagcgaaggttggatgcaccaccttgcgcgccatgcggtcgcatgtttcttgacccgcggcgatctgtacgtgcgctgggaggagggcgccgcggtgttcgacgagctgctcatcgacgcggactgggcggtgaacaacggcaactggatgtggctctcgtgctcgtgcttcttttaccagtacttccgctgctactcgcccgtcgcattcgggcgcaagtacgacccggacggcgcctacgtccggaagtatgtcccggagctcgcccgctttccgaaaaagtacatttacgagccgtggcgcgcgccgatcgccgaccagaataaggctggctgccgcgttggcgtcgactatcccaagccgatcgtgcagcacgacgtggcgtcgaaggagaacatgggcaagttggccgaagcgtacaaggcacacaaggaaagccacgccgacagcggcggcgagcatggttcagagggcaagggcaagggcacgggcaagggcaagggcgcaccgagcaaggcggcgcggggcaaggcacccgccgcgccgccgcccgacgcgaagtcgcgcgcgtcgaagaagcgcaccaggcacagcgagagcgacgacgacgacgacgaagactga

SEQ ID NO: 52 - protein, 581 aa, Diacronema lutheri
MAGSTKTARGAMVVLLWYRKGLRVHDSPALAAACEGATAVCPVFCLDPWFVSSGKVGPIRLRFLAEALADLDASLRARGSRLLVLHGKPEEELPRVAREWGATHIVWEKDGVEPYGLKRDAAVREACAPLGVTITETNGHTICDLDELLKQSKGSPVTTYSTFRTHFDHVVARSPIVLTPTPERIPAPSDAALAEEARGRLSVPSVADIAPSLADAGPSLFPGGEGEALRRLDAHLARDGGAWAGAFEKPKTSPTEIDPFGAGTRSTTVLSAYLKFGCLSPRTFWVRLRDATKGARTRSAPPVSLDGQLLWREFYYACAHAVGPAFGQMEDNPICRQIGWRVPADDPAAAEALAAWRDGRTGYPWIDACMRQLKSEGWMHHLARHAVACFLTRGDLYVRWEEGAAVFDELLIDADWAVNNGNWMWLSCSCFFYQYFRCYSPVAFGRKYDPDGAYVRKYVPELARFPKKYIYEPWRAPIADQNKAGCRVGVDYPKPIVQHDVASKENMGKLAEAYKAHKESHADSGGEHGSEGKGKGTGKGKGAPSKAARGKAPAAPPPDAKSRASKKRTRHSESDDDDDED

SEQ ID NO: 53 - protein, 12 aa, Diacronema lutheri
LYVRWEEGAAVF

SEQ ID NO: 54 - protein, 12 aa, Haematococcus lacustris
LLLPWQWRLKHY

SEQ ID NO: 55 - protein, 12 aa, Nannochloropsis gaditana
LWQSWEERARVF

SEQ ID NO: 56 - protein, 12 aa, Nannochloropsis gaditana
LWQSWEERARVF

SEQ ID NO: 57 - protein, 12 aa, Phaeodactylum tricornutum
LRVDWTKRAEWF

SEQ ID NO: 58 - protein, 12 aa, Phaeodactylum tricornutum
LWQSWEDRATVF

SEQ ID NO: 59 - protein, 12 aa, Diacronema lutheri
LLVDWRHRARWF

SEQ ID NO: 60 - protein, 12 aa, Diacronema lutheri
LYVRWEERAAVF

SEQ ID NO: 61 - DNA, 660 bp, Chaetoceros muelleri
  source 1..660: mol_type = genomic DNA
atgtggagggagtacaattatctcatcggatataccacaccaaatttcgacaaaatggccaataatcctgtagcaaggcaaataccatgggatgatgatccagtcctcttgtcagcttggaagaatgcgcagacagggtatccttatatcgacgccattatgacgcagctgaaacatacaggatggatacatcatttggccagacattcagtcgcttgctttttgacgcgaggagatttgtggcagtcttgggaaaagggggctgaacattttgaagaagagcttattgatgcagattggagcatcaacaattttaattggcagtggttgtcgtgtactgcgcatttttatcagtattttcggtgttacagtcctatatcctttggtaaaaaaacggacaaagacggagcctacatcaaaaaatggttgccacaatttaaggattttccatccaaatatatttatgaaccctggacggcacctcttcatgttcagcagaagtgtggtgtcgtgataggaattgactatccaaaacctatcgttgatcacaaggagataagtaagagtaacatgggacgaatgaagtctgcgtatgatgctcataagactatggaagatgaagttgcttcatctgccaagaaaaaaacaaaaatgaattaa

SEQ ID NO: 62 - protein, 219 aa, Chaetoceros muelleri
MWREYNYLIGYTTPNFDKMANNPVARQIPWDDDPVLLSAWKNAQTGYPYIDAIMTQLKHTGWIHHLARHSVACFLTRGDLWQSWEKGAEHFEEELIDADWSINNFNWQWLSCTAHFYQYFRCYSPISFGKKTDKDGAYIKKWLPQFKDFPSKYIYEPWTAPLHVQQKCGVVIGIDYPKPIVDHKEISKSNMGRMKSAYDAHKTMEDEVASSAKKKTKMN

SEQ ID NO: 63 - protein, 12 aa, Chaetoceros muelleri
LWQSWEKGAEHF

SEQ ID NO: 64 - DNA, 2079 bp, Chaetoceros muelleri
  source 1..2079: mol_type = genomic DNA
atgaatagaatgatattttatcattctccggtacaactgctggcttactgtctcatgattagcagcagcagcagcattcgatcttgccgatcgctagtgcaagggctatcctcctcttcctcccaccaccccttgtcatttcaatggcattctcatgtctgctggtctactactactagtagaagtagaattagtacgtgtgctagaagtcacaaaaacattcacagcaccaagaacgagaaggaacaatcggtagtagtagtagtgtggtttcgagatcatgcccttcgtattcaagataatctagcacttttcaatgctataaatgataataggagacctagtggtaaccatgatgttgatgatgatgatgcttgttggacgtctcgtggtcgtcttattcctgtctttctttggccaaagaatggtggtactaaaagttgtagtactgacagtgctggtggtcaagatcgtccgagtagaggagggagtataacaatggagaaaacgggaggagggacggcaaaagatgtatttgtagtgaatgcattacaaagtttaaatgcaaccttgaatggtaatttatcagtggggatggtagagaatacactgcatgataccgtaagggaactcacagatatttgtcaaagagtcaatgccaacaaggtgtattatctcaagtctcacaaggagaaggaagagtcgatattggaaatgaaattaaaagaaaatgggattgtgcccgtatcatttggtggttcttttagtttgattgattatacaagacatcgagtgccatggaaagaaatcgtaatggaacatccgtggcgatcacctcttattccatttgtagaatatgtccagaaaattatggatgagatgcccaagaagccagtgctgctggacgtatctagagagttgaatcgatacttagttgatgtttcttcaagatatgaatcgtcgtcgatcgtttcaaagccttgcataatagatgatttgaaatcaacagttgggaggacggcgggtggtacaaattggggggaatcaatatctagggcttggcctgcaacagaagaggatgcgaataacgctttgacgtcttttctggattcactgaaaaatccgaatcatcaaaaaagtgatgggggtaatacagaagtcgtagtagaaaaacgtactcatcttgcttctcgtctttcaccatatcttgcaaggggtttgatatctcctggacaagtataccagggcatcaaaagtagtttaggagatgatattgatgtggattcatttttgagaagaatttgttggcgtgattatacgtatgcagcggtacatttatacccaaaagttctccatggggaacccattcgagatggatatgaagagttacaacatggtattccaatggaaaaagatgaacagcggcgtcgactaaaacgttggaaagaaggaaaaacagggtttccgttgattgatgcaggaatgcgccaacttgcaaaagagggttggatgccacagaaagtgagattggcatgtagcacatttttagtggaaggccttggtttgtcttggaaagatgggatgcaacattttgcagagtatcttgtggattttgatgagtcgatcaatagcaacatgtggcagaatgcaggttgtgtgggtctggatccttactatgtgggcatgaattacaaacggcgcatgtattgggatagaaatggagattatgtaagaacatggtgtcccgagctagatctgctgcctgacagcgtggaaattgacatgaggaaaacgagtaaggtagttgattgtttgtacgaaccatggatgtcgccagagcatgtgttggacaaggctggggttgtaatgggaaagacttatccacacagggtttgcaacgatagggaaacgaggtctacatttttttctcgtgtgagagacatcaggttgaaatggcctgcaacaaagattgatgctcagaaacgagatttagtgtgcttgggatctgcaggatatgttggtctcttcactccaagagcattgcagatacgggaatcatcagtctattcctctaattaa

SEQ ID NO: 65 - protein, 692 aa, Chaetoceros muelleri
MNRMIFYHSPVQLLAYCLMISSSSSIRSCRSLVQGLSSSSSHHPLSFQWHSHVCWSTTTSRSRISTCARSHKNIHSTKNEKEQSVVVVVWFRDHALRIQDNLALFNAINDNRRPSGNHDVDDDDACWTSRGRLIPVFLWPKNGGTKSCSTDSAGGQDRPSRGGSITMEKTGGGTAKDVFVVNALQSLNATLNGNLSVGMVENTLHDTVRELTDICQRVNANKVYYLKSHKEKEESILEMKLKENGIVPVSFGGSFSLIDYTRHRVPWKEIVMEHPWRSPLIPFVEYVQKIMDEMPKKPVLLDVSRELNRYLVDVSSRYESSSIVSKPCIIDDLKSTVGRTAGGTNWGESISRAWPATEEDANNALTSFLDSLKNPNHQKSDGGNTEVVVEKRTHLASRLSPYLARGLISPGQVYQGIKSSLGDDIDVDSFLRRICWRDYTYAAVHLYPKVLHGEPIRDGYEELQHGIPMEKDEQRRRLKRWKEGKTGFPLIDAGMRQLAKEGWMPQKVRLACSTFLVEGLGLSWKDGMQHFAEYLVDFDESINSNMWQNAGCVGLDPYYVGMNYKRRMYWDRNGDYVRTWCPELDLLPDSVEIDMRKTSKVVDCLYEPWMSPEHVLDKAGVVMGKTYPHRVCNDRETRSTFFSRVRDIRLKWPATKIDAQKRDLVCLGSAGYVGLFTPRALQIRESSVYSSN

SEQ ID NO: 66 - protein, 12 aa, Chaetoceros muelleri
LGLSWKDGMQHF

SEQ ID NO: 67 - DNA, 1893 bp, Chaetoceros muelleri
  source 1..1893: mol_type = genomic DNA
atgaaaaagggcacaagaacaaatagccataaagatgacaatctaagggtgacagatactactcagcaggaagaaagagttcgactggtttggcacagacgtgatctccgtttacatgataatgaattatatgctgacgacgattcctacaggaaccaccaccacagcaattgctgctactttgatcctcgtgagaagcctcccggctccaccaagaacaggaggaatgattcatccttgaaaatcataagtctctttgtctttgacaatcaccattttcaaccccaaccgtcctcgattggaggagaagagaagaaatttcatacaatttggtgtggtcctcactatacaagcgcattaatagacgccgttgattctctccgaagtagtatccaattgctcggaggagaattgcttgtccgtgtgggagatcctattgtgattgttcctcaaattgcgctgcaaattggagcgacggaagtatggtacagtgaagaacctggtacatatgagtgtcaagttgcaaagaatatccaacaggtctgcacccttcagtatggcatcaaagtttgtagcaaagttggatatacactctatcatcccaatgatttgccttggaatcacaatgaatggagtcagttggctcatccaaagaataaacaaaagaaaaagaacaagagaacaacagaaaaacaggagacacacttgaaaacgttcttggaggaatcagtcgttgatgttagttgtgatcgatttacgggtatgtgtcgaataatgggtgattttcgaagagctgtcacgagttatgcctccgttcgaccaattatcccagcaccgacagaacttttgaaaccaactgggtacgatttactgaatatagaccaggggaggatacccacattggaggacttgattcattccatcatacaggagaataatgacgcaacttcaaaaattagcatcatgggcatggatgacgagactattcagtttgtcctaaaatcagccattgaagagcgaaatgttagacataaccagagacacgtttctggtggataccacctgtgtggagaattggcagcactacaaaggttggaaacattcattggaaatggatacgccaaaatagcaaatcgaagtttggcagatgtatccaaccataatagttcaagactctccacatactttgcacttggaactctctcaccacggacagtttattggagggcacacgctgcaggggaaggttgtgagtggctcaagagtcatttggaaatgcgtgattttttcctatttacgtgctttgcagcaggatccaacttattccaagaaaatggtatgccattaagcagtgcaagtaagaaaaaagagcacttcatccagtggaatgatccgactgatgcagcccatttgcaaaagtggaaacaatgggcagcaggaaaaacacaattaccattgattgacgctggcatgaaagaacttttgtctactgggtattgttccaaccgtgtacgacaaaatatggcaagtgtactgacaaaagatttgcacttggattggagagcaggggctgaatggttccaatttttactagaagatcattgtgttggatccaattatggcaattggttgtatttctcaggtgtaggtcctgatccaaagaatcgacattttcgaacggtctctcagatgaaaaagtatgatccaaaggggcactacataaagaaatggatcccagaactaagcaatgttgattgcgtggaagttttgtttcgaccctgggactttgggattgcttcgtttcagtctccaattgtagatccatcgtctcagtatacttggcaagactggaaagatattcaacaaacgggtgggcttaattcggaggaataa

SEQ ID NO: 68 - protein, 630 aa, Chaetoceros muelleri
MKKGTRTNSHKDDNLRVTDTTQQEERVRLVWHRRDLRLHDNELYADDDSYRNHHHSNCCYFDPREKPPGSTKNRRNDSSLKIISLFVFDNHHFQPQPSSIGGEEKKFHTIWCGPHYTSALIDAVDSLRSSIQLLGGELLVRVGDPIVIVPQIALQIGATEVWYSEEPGTYECQVAKNIQQVCTLQYGIKVCSKVGYTLYHPNDLPWNHNEWSQLAHPKNKQKKKNKRTTEKQETHLKTFLEESVVDVSCDRFTGMCRIMGDFRRAVTSYASVRPIIPAPTELLKPTGYDLLNIDQGRIPTLEDLIHSIIQENNDATSKISIMGMDDETIQFVLKSAIEERNVRHNQRHVSGGYHLCGELAALQRLETFIGNGYAKIANRSLADVSNHNSSRLSTYFALGTLSPRTVYWRAHAAGEGCEWLKSHLEMRDFFLFTCFAAGSNLFQENGMPLSSASKKKEHFIQWNDPTDAAHLQKWKQWAAGKTQLPLIDAGMKELLSTGYCSNRVRQNMASVLTKDLHLDWRAGAEWFQFLLEDHCVGSNYGNWLYFSGVGPDPKNRHFRTVSQMKKYDPKGHYIKKWIPELSNVDCVEVLFRPWDFGIASFQSPIVDPSSQYTWQDWKDIQQTGGLNSEE

SEQ ID NO: 69 - protein, 12 aa, Chaetoceros muelleri
LHLDWRAGAEWF

SEQ ID NO: 70 - DNA, 660 bp, Chaetoceros gracilis
  source 1..660: mol_type = genomic DNA
atgtggagggagtacaattatctcatgggatataccacaccaaatttcgacaaaatggccaataatcccgtagcaaggcaaataccatgggatgacgatccagtcctcttgtcagcttggaagaatgcgcagacaggatatccttatattgacgctattatgacgcagctgaaacatacaggatggatacatcatttggccagacattcagtcgcttgctttttgacgcgaggagatttgtggcagtcttgggaaaagggggctgaacattttgaagaagagcttattgatgcagattggagcatcaacaattttaattggcagtggttgtcgtgcactgcgcatttttatcagtattttcggtgttacagtcctatatcctttggtaaaaaaacggataaagacggagcctacatcaaaaaatggttgccacaatttaaggattttccatccaaatatatttatgaaccctggacggcacctcttcatgttcagcagaagtgtggtgtcgtgataggaattgactatccaaaacctatcgttgatcacaaggagataagcaagagtaacatgggacgaatgaagtctgcttacgatgctcataaggctatggaagataaagttgcttcatctgccaggaaaaaaacaaaattgaattaa

SEQ ID NO: 71 - protein, 219 aa, Chaetoceros gracilis
MWREYNYLMGYTTPNFDKMANNPVARQIPWDDDPVLLSAWKNAQTGYPYIDAIMTQLKHTGWIHHLARHSVACFLTRGDLWQSWEKGAEHFEEELIDADWSINNFNWQWLSCTAHFYQYFRCYSPISFGKKTDKDGAYIKKWLPQFKDFPSKYIYEPWTAPLHVQQKCGVVIGIDYPKPIVDHKEISKSNMGRMKSAYDAHKAMEDKVASSARKKTKLN

SEQ ID NO: 72 - protein, 12 aa, Chaetoceros gracilis
LWQSWEKGAEHF

SEQ ID NO: 73 - DNA, 1308 bp, Chaetoceros gracilis
  source 1..1308: mol_type = genomic DNA
atggcagataaggtaaatgtgttttggtttagaagagatttacgtttggacgataatgtaggcttttacaaggcattgaatggcagccatcccgtactacccattttcatattcgataaaaacattttagaagaactacctgaagacgatgctcgcgtaacattcattttcgatactctccaaaaaatgcgagatgaacttcaggagaacggatgtagcttggcgatgtatcacggcacaccagaaaaagtatttaaatcgcttctctcagactttgatgtgcagaacgtcattaccaaccacgattacgaaccttatgccaaagaacgagatgaggaaatttcaaaaatgctgaaagaaaaagaggtgggtttctacacctttaaagaccaggttatttacgaaaaggacgaggtggtaaaagatgatggcgacccatatgtggtgtacactccttatatgaaaaagtggaaagaaacttttaaaaaagacggtgacgatgtcaagatttattacacgtcgcaggtcatggacaacttagtgcaacattcacgtttgcccaatcttagcctgagcgatatggggtttaaacgttcaaaaattgaagttcccgattacgacgttaccccaaccactattcaagagtatgaaaaaacaagaaattttcctgcgaaacaaggcacttcacgtttggggccacacttgcgctttggaactgtaagcgttcgcaaaatggtaaaaaaagcgattgccgaaaaaaatgaaaccttttgggaggaattgatatggcgcgaattttttatgcagatattatggcactttcccgaaacggttgataccgcttttcgaaaaaaatacgatcgcgttccttggcgaaaagccaaagctgatttcaaaaaatggaaagaaggaaaaacgggatttcctttggttgatgctggtatgcggcaacttaatgaaactgggtacatgcacaaccgagtcagaatgttggtagccagtttcttatgcaaacacctattaatcgattggcgttggggtgaagcctatttcgctgaaaaattactggattatgaactttccagcaatgtgggcaattggcagtgggctgccggaagtggtgtggatgctgctccctatttcagaattttcaatccgaccacccaaatagagaaattcgataaagacaaaaaatatatcaagaaatgggtaccagaatacaataccgaagactatccaaaaaaaatggtagaccataaagaagcaagagaaagagcattggacacttataagaaggcaataaattaa

SEQ ID NO: 74 - protein, 435 aa, Chaetoceros gracilis
MADKVNVFWFRRDLRLDDNVGFYKALNGSHPVLPIFIFDKNILEELPEDDARVTFIFDTLQKMRDELQENGCSLAMYHGTPEKVFKSLLSDFDVQNVITNHDYEPYAKERDEEISKMLKEKEVGFYTFKDQVIYEKDEVVKDDGDPYVVYTPYMKKWKETFKKDGDDVKIYYTSQVMDNLVQHSRLPNLSLSDMGFKRSKIEVPDYDVTPTTIQEYEKTRNFPAKQGTSRLGPHLRFGTVSVRKMVKKAIAEKNETFWEELIWREFFMQILWHFPETVDTAFRKKYDRVPWRKAKADFKKWKEGKTGFPLVDAGMRQLNETGYMHNRVRMLVASFLCKHLLIDWRWGEAYFAEKLLDYELSSNVGNWQWAAGSGVDAAPYFRIFNPTTQIEKFDKDKKYIKKWVPEYNTEDYPKKMVDHKEARERALDTYKKAIN

SEQ ID NO: 75 - protein, 12 aa, Chaetoceros gracilis
LLIDWRWGEAYF

SEQ ID NO: 76 - DNA, 2100 bp, Chaetoceros gracilis
  source 1..2100: mol_type = genomic DNA
atgaaaagaatgatattttatcattctccggtacaactgctggcttactgtctcatgattagcagcagcagcagcagcagcattcgatcttgccgatcgctagtacaaggactatcctcctcttcctcccgcctcctatcatttcaatggcattctcatgtctgctggtctactactactactactagaagtagaattagtacgtgtactagaagtcacaaaaacattcacaacaccaagaacgagaaggaacaatcggtagtcgtagtgtggtttcgagatcatgcccttcgtatacaagataatctagcacttgtcactgctataaatgataatagggggcggcctactagtagtgataaccatgatgttgtcgaggatgatgatgatgacgatgcttgctggacatctcttggtctcattcctgtctttctttggccaaagaatggtggtactaaaagttgtagtactgacagcgctggtggtcaagatcgtccaagtagaggagggagtataataatggagaaaacggaaggagggacggcaaaagatgtatttgttgtgaatgcattacaaagtttaaatgcaaccttgaatggcaatttatcagtggggatggtagagaatacactgcatgataccgcaagggaactcacagatatttgtcaaagagtcaatgccaacaaggtgtattatctcaagtctcacaaggagatggaagagtcgatattggaaatgaaattaaaagaaaatgggattgtgcctgtatcatttggtggttgttatagtttgattgattatgcaagacatcaagtgccatggaaagacatcgtaatggaacatccgtggcgatcacctcttattccatttgtagaatatgtcaagaaaattatggatgagatgcccaagaagccagtgctgctggacgtacctagagagttaaatcgatacttaggtgatgtttcttcaagatgtgagtcgtcgtcaatcgtttcaaagccttgcataatagatgatttgaaatcaacagttggaaggacagagggtggtacaaattgggggaaatcaatatctagggcttggcctgcctcagaagaggatgcgaataacgctttaacgtgttttctggattcactgaaagatccgaatcatcaaaaaagtaatgggggtaatacagaagtcgtagtagaaaaacgtacacatcttgcttctcgtctttcaccatatcttgcaaggggtttgatatctcctggacaagtataccagggcatcaaaagtagtttaggagatgatattgatgtggattcatttttgagaagaatttgttggcgtgattatacgtatgcagcggtacatttatacccaaaggttctgcatggggaacccattcgagatggatatgaagagttacaagatggtatactaatggaaaaagatgaacaacagcgtagactaaaatgttggaaagaagggaaaacagggtttccgttgattgatgcaggaatgcgccaacttgcaaaagagggttggatgccacagaaagtgagactggcatgtagcacatttttagtggaaggccttggtttgtcttggaaagatgggatgcaacattttgcagagtatcttgtggattttgatgagtcgatcaatagcaacatgtggcagaatgcaggttgtgtaggtctggatccttactatgtgggcatgaattacaaacggcgcatgtattgggatagaactggagattatgtaagaacatggtgtcccgaacttgatctgctgcctgatagcgtggaaattgatatggggaaaacgagcaaggtagttgattgtttgtacgaaccatggatgtcaccagagcatgtgttagacaaggctgggattgtaatgggagagacgtatccaaacagggtttgcaacgatagggaaacgaggtctacatttttttctcgtgtgagagacatcaggttgaaatggcctgcaacaaagattgatgctcagaaacgagatttagtgcgcttgggatctgcaggagatgttggtctcttcactccaagagctttgcagatacgggaatcatcggtatattcctctaattag

SEQ ID NO: 77 - protein, 699 aa, Chaetoceros gracilis
MKRMIFYHSPVQLLAYCLMISSSSSSSIRSCRSLVQGLSSSSSRLLSFQWHSHVCWSTTTTTRSRISTCTRSHKNIHNTKNEKEQSVVVVWFRDHALRIQDNLALVTAINDNRGRPTSSDNHDVVEDDDDDDACWTSLGLIPVFLWPKNGGTKSCSTDSAGGQDRPSRGGSIIMEKTEGGTAKDVFVVNALQSLNATLNGNLSVGMVENTLHDTARELTDICQRVNANKVYYLKSHKEMEESILEMKLKENGIVPVSFGGCYSLIDYARHQVPWKDIVMEHPWRSPLIPFVEYVKKIMDEMPKKPVLLDVPRELNRYLGDVSSRCESSSIVSKPCIIDDLKSTVGRTEGGTNWGKSISRAWPASEEDANNALTCFLDSLKDPNHQKSNGGNTEVVVEKRTHLASRLSPYLARGLISPGQVYQGIKSSLGDDIDVDSFLRRICWRDYTYAAVHLYPKVLHGEPIRDGYEELQDGILMEKDEQQRRLKCWKEGKTGFPLIDAGMRQLAKEGWMPQKVRLACSTFLVEGLGLSWKDGMQHFAEYLVDFDESINSNMWQNAGCVGLDPYYVGMNYKRRMYWDRTGDYVRTWCPELDLLPDSVEIDMGKTSKVVDCLYEPWMSPEHVLDKAGIVMGETYPNRVCNDRETRSTFFSRVRDIRLKWPATKIDAQKRDLVRLGSAGDVGLFTPRALQIRESSVYSSN

SEQ ID NO: 78 - protein, 12 aa, Chaetoceros gracilis
LGLSWKDGMQHF

SEQ ID NO: 79 - protein, 12 aa, Chaetoceros muelleri
LWQSWEKRAEHF

SEQ ID NO: 80 - protein, 12 aa, Chaetoceros muelleri
LGLSWKDRMQHF

SEQ ID NO: 81 - protein, 12 aa, Chaetoceros muelleri
LHLDWRARAEWF

SEQ ID NO: 82 - protein, 12 aa, Chaetoceros gracilis
LWQSWEKRAEHF

SEQ ID NO: 83 - protein, 12 aa, Chaetoceros gracilis
LLIDWRWREAYF

SEQ ID NO: 84 - protein, 12 aa, Chaetoceros gracilis
LGLSWKDRMQHF

SEQ ID NO: 85 - DNA, 1560 bp, Cyanidioschyzon merolae
  source 1..1560: mol_type = genomic DNA
atgtgggtcatcttgaccatggcaagtgcagttcactggttccgaaagggtctgcgcttgcacgacaaccctgccctgcttgatgcggtgcaaaatcccaccacaacgtacgtgttgccagtattctgccttgacccgatattcctgcgacccgagactgtgggcgtgaaccgcatgaactttctgctagagtgcttacaggatctggaccagcaacttcgcaagctgcactctagactgtttgtgcttcggggcaatccgctggagcaactacccgtctttttccgaaagtatcatacgcgcttgctgacgttcgagttcgacacagagccgtatgcgaagcagcgagacacacaggttcggcgactctgtgccgagctgggcatcgaggtgcgcactcgtgcgacgcacacgctctacgatcccgaggatattcgacgtgaactcggagatcgtcccacaccgcttacctacaaaagcttctacgcgttcgtaacggagcgtctgggccagccgatgagtgcgctggacgcacccgcgcctgcgagcggtttccaaacacccgatgtggacctggacacctacaccgttccgtcgctttcggagctggaggcgtatcagggcctcgaagtggagacacctttccgcggtggcgagactgaagcactcaggcgcatggagaactttttacgagaacgggcggatgaagttcgctcgttcgcgaaacccgcgacatcgccaacggcatggccagtagcatccacgacgcaactgtcgccgtacttcaagttcggctgcctatcgccgcggctctttgtcgagcgcgtccgctcactacgaccgctccagcaaccaccggtctctctgattggacagatctggtggcgggaattcttcacatacgtcgcctatgtgacgccgcactttcatcaaatgcaggggaatcctatctgtcgacagataccgtggcgagaagctgcagatgatgcacgctatagggcgtgggaggaggctcgaaccggatacccctggatcgatgcttgcatggtgcagctgcgacaggagggctggctgcaccatctcgcacgacacgctgtcgcttgtttcctgacacggggtgacctctgggtcagctgggaacgaggtcgtgagacctttgatcgtctgttggtagacgccgactacagtctgaacaatgcaaattggttatggttgtcaagctcagcattttttcatcagtactatcgcgtctattctccgatcagtttcccccaaaagtacgatccaaatggtgaatatgtgcgacattttctgccagtgttgaaggagatgccgtcaaaatacatttacaccccgtggttagcaccagttgtggtgcagaaaaaggccaaatgcatcattggtgaggactatccgcatccgatcgtggatcatgcagtcgttatgcgagagaatatgaggcgcatgcgcgaggcacttgacgcgggcgctccgcagcgtgttccgaagcggccacgacgcgatgccaacgaagcatcgtcatcgtcatcgtcgtcatag

SEQ ID NO: 86 - protein, 519 aa, Cyanidioschyzon merolae
MWVILTMASAVHWFRKGLRLHDNPALLDAVQNPTTTYVLPVFCLDPIFLRPETVGVNRMNFLLECLQDLDQQLRKLHSRLFVLRGNPLEQLPVFFRKYHTRLLTFEFDTEPYAKQRDTQVRRLCAELGIEVRTRATHTLYDPEDIRRELGDRPTPLTYKSFYAFVTERLGQPMSALDAPAPASGFQTPDVDLDTYTVPSLSELEAYQGLEVETPFRGGETEALRRMENFLRERADEVRSFAKPATSPTAWPVASTTQLSPYFKFGCLSPRLFVERVRSLRPLQQPPVSLIGQIWWREFFTYVAYVTPHFHQMQGNPICRQIPWREAADDARYRAWEEARTGYPWIDACMVQLRQEGWLHHLARHAVACFLTRGDLWVSWERGRETFDRLLVDADYSLNNANWLWLSSSAFFHQYYRVYSPISFPQKYDPNGEYVRHFLPVLKEMPSKYIYTPWLAPVVVQKKAKCIIGEDYPHPIVDHAVVMRENMRRMREALDAGAPQRVPKRPRRDANEASSSSSSS

SEQ ID NO: 87 - DNA, 2178 bp, Cyanidioschyzon merolae
  source 1..2178: mol_type = genomic DNA
atgcaccattgtgtcacagtgaacggcagctcgttgctgttttgcgaagtgattccgaggtctacatatggctggtgccctggtgagcgctactgcagtgacagtcagggtttcacggcacagagggacttggttgacgctcgcccgagatcgtacaacgggcgacggacaccgagccggtatcgcgctcttctacgcatgcgaaaagcaaagcgtcggcccgttgagtcctctaatcgagcaacggattcacctgatacgttgttctcaaaaatagacgcacagaaaacggccgtgaagcgatcatcatcctcagcagctaccatcgtgtggctccgaggacgcggggacctgcgaatacacgataatccgttattgctgcaagcgcagaggctcaatgaacctcttttcataatgtttacatggtcatcggcggatgcggacaaaaactacggctttggtgaagcacaacgcgttttcctcttcagcgccgtggatgcactcaatcgagccttaaacatgcgctttcagcaggtgattcactacgtgcgtctcagcgatgacgcaggcctcgaagagtacctgcaattgtttcatttccttgaagcctctttgtcagcacgaacgctgctgatggctcgacgctatgagcctcctctactccagctcgacatggagctggaatgcacgctcacaaaacagcgtaaatggaaggtgtatacgcacaacatgcacctcctacatgagccctggacagtagcgtacgatggcgatgcaacctcgagtgctggacactttggaacactgcttcccttctggcaggcctggcaacgaaacgccgacctaccgcccgagcctgcagcagcgccgtctacgctaccgccggctgcggcgctggagcgctgcgagccacggacaccagcatgctgtgagaagccgcctccgcttgctggagatgcgtttgtcgataggacaacacgctgcgcgcccttccagtttgtcacatcgttggtggaaacggggttgcacccggtgcgtccgggtacaaaacgctgggatacggtgctgctcggttcgtgggcggtcgacgaggaacgcgttcgcgcgtttttgcgggattttctggaacaccgactacccctgtacgagaagaacaaatctagagcagacctcgaggtcgtatcgcgtctgtcaccgtatctggcactgggtatgctcagcgcacgggaggtgttccacgctacgagagcggcctctagacgactggcggcatcaaagcgatccaagacatttgagcgtcgacttatctggcgagacctggcgtactggacgctctatatgtttccagaggcggtcacgacgcccattcggagccattatgcctcgcaggaatggaacgaggatccgcgtctgctcgcggcctggcagcggggatccacgggataccccatcattgatgccggaatgcgacaactttggcaaacgggttggatgccccagaatatccgcatggctgcggcatcgtttctggtcgagtacctcaatatacactggatacacggcctgcaatggttccatcgtacgctcatcgatttggacattgccatcaacgcgatgatgtggcagaatgcgggacgcaccggcctggacatgtggaatttcgttattcatccagagaccagcgcccggtcgagcgacccaactggtgcgtacgttcgcaagtggctacccgaactagctcaactgccgaacgcttatattcatgcaccgtggaaagcgcctgagtcggtcttgtccagtgcaggcgttcagcttggtgcgacctacccccagcgcatcatcgctgaccttggagcagctcggaaacaatcgcaagcggcagttctcgagatgcgatctcgatccatgccccagtttttcaacgctgacggttacgatcgaatacgggtacccgtcctgaaagccgtctcattgccgcatgaaagattccagcagacagcgacagcggataacacggtttggcggcatgtgtttactcgacgcgagtttcgcgaggccccctttgcgacgcacctgccacatgaaacagaagcgtgtgatcggcaggaggcgcagttgctcccgaaggactccacgcgggccatgcaaggcaaaagtgacgctcaagctgctgcctga

SEQ ID NO: 88 - protein, 725 aa, Cyanidioschyzon merolae
MHHCVTVNGSSLLFCEVIPRSTYGWCPGERYCSDSQGFTAQRDLVDARPRSYNGRRTPSRYRALLRMRKAKRRPVESSNRATDSPDTLFSKIDAQKTAVKRSSSSAATIVWLRGRGDLRIHDNPLLLQAQRLNEPLFIMFTWSSADADKNYGFGEAQRVFLFSAVDALNRALNMRFQQVIHYVRLSDDAGLEEYLQLFHFLEASLSARTLLMARRYEPPLLQLDMELECTLTKQRKWKVYTHNMHLLHEPWTVAYDGDATSSAGHFGTLLPFWQAWQRNADLPPEPAAAPSTLPPAAALERCEPRTPACCEKPPPLAGDAFVDRTTRCAPFQFVTSLVETGLHPVRPGTKRWDTVLLGSWAVDEERVRAFLRDFLEHRLPLYEKNKSRADLEVVSRLSPYLALGMLSAREVFHATRAASRRLAASKRSKTFERRLIWRDLAYWTLYMFPEAVTTPIRSHYASQEWNEDPRLLAAWQRGSTGYPIIDAGMRQLWQTGWMPQNIRMAAASFLVEYLNIHWIHGLQWFHRTLIDLDIAINAMMWQNAGRTGLDMWNFVIHPETSARSSDPTGAYVRKWLPELAQLPNAYIHAPWKAPESVLSSAGVQLGATYPQRIIADLGAARKQSQAAVLEMRSRSMPQFFNADGYDRIRVPVLKAVSLPHERFQQTATADNTVWRHVFTRREFREAPFATHLPHETEACDRQEAQLLPKDSTRAMQGKSDAQAAA